European Patent Application EP 4 455 165 A1, published October 30, 2024. Title: 双特异性抗体及其应用. Applicant: 广州爱思迈生物医药科技有限公司. Application CN. The sequence listing filed with the application follows.

SEQUENCE LISTING (168 sequences)

SEQ ID NO: 1 - protein, 98 aa, synthetic construct
  source 1..98: note = 7D5 CH1
ASTKGPSVFPLAPSSKSTSGGTAALGCLVKDYFPEPVTVSWNSGALTSGVHTFPAVLQSSGLYALYSVVTVPSSSLGTQTYICNVNHKPSNTKVDKKV

SEQ ID NO: 2 - DNA, 294 bp, synthetic construct
  source 1..294: mol_type = other DNA; note = 7D5 CH1
gctagcaccaagggcccatcggtcttccccctggcaccctcctccaagagcacctctgggggcacagcggccctgggctgcctggtcaaggactacttccccgaaccggtgacggtgtcgtggaactcaggcgccctgaccagcggcgtgcacaccttcccggctgtcctacagtcctcaggactctacgcgctctatagcgttgtgaccgtgccctccagcagcttgggcacccagacctacatctgcaacgtgaatcacaagcccagcaacaccaaggtggacaagaaagtt

SEQ ID NO: 3 - protein, 106 aa, synthetic construct
  source 1..106: note = 7D5 CL
TVAAPSVFIFPPSDEQLKSGTASVVCLLNNFYPREAKVQWKVDNALQSGNSQESVTEQDSKDSTYSLMSMLTLSKADYEKHKVYACEVTHQGLSSPVTKSFNRGEC

SEQ ID NO: 4 - DNA, 318 bp, synthetic construct
  source 1..318: mol_type = other DNA; note = 7D5 CL
actgtcgcagctccatccgtgttcatctttccaccctccgacgagcaactgaaaagtggcacagcctccgtcgtctgtctgctgaacaatttctaccctcgggaggccaaggtccagtggaaggtggacaacgctctccagagtggaaatagccaagagtccgttactgaacaggactctaaggattcaacctacagtctcatgagcatgctgactctgagcaaggcagattatgagaagcacaaagtctacgcatgtgaagtgactcatcagggactcagctcacccgttaccaagtctttcaacaggggagagtgt

SEQ ID NO: 5 - protein, 98 aa, synthetic construct
  source 1..98: note = 7D10 CH1
ASTKGPSVFPLAPSSKSTSGGTAALGCLVKDYFPEPVTVSWNSGALTSGVHTFPAVLQSSGLYTLMSTVTVPSSSLGTQTYICNVNHKPSNTKVDKKV

SEQ ID NO: 6 - DNA, 294 bp, synthetic construct
  source 1..294: mol_type = other DNA; note = 7D10 CH1
gctagcaccaagggcccatcggtcttccccctggcaccctcctccaagagcacctctgggggcacagcggccctgggctgcctggtcaaggactacttccccgaaccggtgacggtgtcgtggaactcaggcgccctgaccagcggcgtgcacaccttcccggctgtcctacagtcctcaggactctacacgctcatgagcacggtgaccgtgccctccagcagcttgggcacccagacctacatctgcaacgtgaatcacaagcccagcaacaccaaggtggacaagaaagtt

SEQ ID NO: 7 - protein, 106 aa, synthetic construct
  source 1..106: note = 7D10 CL
TVAAPSVFIFPPSDEQLKSGTASVVCLLNNFYPREAKVQWKVDNALQSGNSQESVTEQDSKDSTYFLLSMLTLSKADYEKHKVYACEVTHQGLSSPVTKSFNRGEC

SEQ ID NO: 8 - DNA, 318 bp, synthetic construct
  source 1..318: mol_type = other DNA; note = 7D10 CL
actgtcgcagctccatccgtgttcatctttccaccctccgacgagcaactgaaaagtggcacagcctccgtcgtctgtctgctgaacaatttctaccctcgggaggccaaggtccagtggaaggtggacaacgctctccagagtggaaatagccaagagtccgttactgagcaggactctaaggattcaacctactttctcctgagcatgctgactctgagcaaggcagattatgagaagcacaaagtctacgcatgtgaagtgactcatcagggactcagctcacccgttaccaagtctttcaacaggggagagtgt

SEQ ID NO: 9 - protein, 98 aa, synthetic construct
  source 1..98: note = 7D11 CH1
ASTKGPSVFPLAPSSKSTSGGTAALGCLVKDYFPEPVTVSWNSGALTSGVHTFPAVLQSSGLYELTSIVTVPSSSLGTQTYICNVNHKPSNTKVDKKV

SEQ ID NO: 10 - DNA, 294 bp, synthetic construct
  source 1..294: mol_type = other DNA; note = 7D11 CH1
gctagcaccaagggcccatcggtcttccccctggcaccctcctccaagagcacctctgggggcacagcggccctgggctgcctggtcaaggactacttccccgaaccggtgacggtgtcgtggaactcaggcgccctgaccagcggcgtgcacaccttcccggctgtcctacagtcctcaggactctacgagctcacgagcattgtgaccgtgccctccagcagcttgggcacccagacctacatctgcaacgtgaatcacaagcccagcaacaccaaggtggacaagaaagtt

SEQ ID NO: 11 - protein, 106 aa, synthetic construct
  source 1..106: note = 7D11 CL
TVAAPSVFIFPPSDEQLKSGTASVVCLLNNFYPREAKVQWKVDNALQSGNSQESVTEQDSKDSTYFLSSYLTLSKADYEKHKVYACEVTHQGLSSPVTKSFNRGEC

SEQ ID NO: 12 - DNA, 318 bp, synthetic construct
  source 1..318: mol_type = other DNA; note = 7D11 CL
actgtcgcagctccatccgtgttcatctttccaccctccgacgagcaactgaaaagtggcacagcctccgtcgtctgtctgctgaacaatttctaccctcgggaggccaaggtccagtggaaggtggacaacgctctccagagtggaaatagccaagagtccgttactgagcaggactctaaggattcaacctactttctcagtagctatctgactctgagcaaggcagattatgagaagcacaaagtctacgcatgtgaagtgactcatcagggactcagctcacccgttaccaagtctttcaacaggggagagtgt

SEQ ID NO: 13 - protein, 98 aa, synthetic construct
  source 1..98: note = 7F4 CH1
ASTKGPSVFPLAPSSKSTSGGTAALGCLVKDYFPEPVTVSWNSGALTSGVHTFPAVLQSSGLYQLFSTVTVPSSSLGTQTYICNVNHKPSNTKVDKKV

SEQ ID NO: 14 - DNA, 294 bp, synthetic construct
  source 1..294: mol_type = other DNA; note = 7F4 CH1
gctagcaccaagggcccatcggtcttccccctggcaccctcctccaagagcacctctgggggcacagcggccctgggctgcctggtcaaggactacttccccgaaccggtgacggtgtcgtggaactcaggcgccctgaccagcggcgtgcacaccttcccggctgtcctacagtcctcaggactctaccagctctttagcacggtgaccgtgccctccagcagcttgggcacccagacctacatctgcaacgtgaatcacaagcccagcaacaccaaggtggacaagaaagtt

SEQ ID NO: 15 - protein, 106 aa, synthetic construct
  source 1..106: note = 7F4 CL
TVAAPSVFIFPPSDEQLKSGTASVVCLLNNFYPREAKVQWKVDNALQSGNSQESVTEQDSKDSTYFLYSLLTLSKADYEKHKVYACEVTHQGLSSPVTKSFNRGEC

SEQ ID NO: 16 - DNA, 318 bp, synthetic construct
  source 1..318: mol_type = other DNA; note = 7F4 CL
actgtcgcagctccatccgtgttcatctttccaccctccgacgagcaactgaaaagtggcacagcctccgtcgtctgtctgctgaacaatttctaccctcgggaggccaaggtccagtggaaggtggacaacgctctccagagtggaaatagccaagagtccgttactgagcaggactctaaggattcaacctactttctctatagcctgctgactctgagcaaggcagattatgagaagcacaaagtctacgcatgtgaagtgactcatcagggactcagctcacccgttaccaagtctttcaacaggggagagtgt

SEQ ID NO: 17 - protein, 98 aa, synthetic construct
  source 1..98: note = 7F10 CH1
ASTKGPSVFPLAPSSKSTSGGTAALGCLVKDYFPEPVTVSWNSGALTSGVHTFPAVLQSSGLYMLTSWVTVPSSSLGTQTYICNVNHKPSNTKVDKKV

SEQ ID NO: 18 - DNA, 294 bp, synthetic construct
  source 1..294: mol_type = other DNA; note = 7F10 CH1
gctagcaccaagggcccatcggtcttccccctggcaccctcctccaagagcacctctgggggcacagcggccctgggctgcctggtcaaggactacttccccgaaccggtgacggtgtcgtggaactcaggcgccctgaccagcggcgtgcacaccttcccggctgtcctacagtcctcaggactctacatgctcacgagctgggtgaccgtgccctccagcagcttgggcacccagacctacatctgcaacgtgaatcacaagcccagcaacaccaaggtggacaagaaagtt

SEQ ID NO: 19 - protein, 106 aa, synthetic construct
  source 1..106: note = 7F10 CL
TVAAPSVFIFPPSDEQLKSGTASVVCLLNNFYPREAKVQWKVDNALQSGNSQESVTEQDSKDSTYNLASTLTLSKADYEKHKVYACEVTHQGLSSPVTKSFNRGEC

SEQ ID NO: 20 - DNA, 318 bp, synthetic construct
  source 1..318: mol_type = other DNA; note = 7F10 CL
actgtcgcagctccatccgtgttcatctttccaccctccgacgagcaactgaaaagtggcacagcctccgtcgtctgtctgctgaacaatttctaccctcgggaggccaaggtccagtggaaggtggacaacgctctccagagtggaaatagccaagagtccgttactgagcaggactctaaggattcaacctacaatctcgctagcacgctgactctgagcaaggcagattatgagaagcacaaagtctacgcatgtgaagtgactcatcagggactcagctcacccgttaccaagtctttcaacaggggagagtgt

SEQ ID NO: 21 - protein, 98 aa, synthetic construct
  source 1..98: note = 7G1 CH1
ASTKGPSVFPLAPSSKSTSGGTAALGCLVKDYFPEPVTVSWNSGALTSGVHTFPAVLQSSGLYSLYSMVTVPSSSLGTQTYICNVNHKPSNTKVDKKV

SEQ ID NO: 22 - DNA, 294 bp, synthetic construct
  source 1..294: mol_type = other DNA; note = 7G1 CH1
gctagcaccaagggcccatcggtcttccccctggcaccctcctccaagagcacctctgggggcacagcggccctgggctgcctggtcaaggactacttccccgaaccggtgacggtgtcgtggaactcaggcgccctgaccagcggcgtgcacaccttcccggctgtcctacagtcctcaggactctactcgctctatagcatggtgaccgtgccctccagcagcttgggcacccagacctacatctgcaacgtgaatcacaagcccagcaacaccaaggtggacaagaaagtt

SEQ ID NO: 23 - protein, 106 aa, synthetic construct
  source 1..106: note = 7G1 CL
TVAAPSVFIFPPSDEQLKSGTASVVCLLNNFYPREAKVQWKVDNALQSGNSQESVTEQDSKDSTYMLISILTLSKADYEKHKVYACEVTHQGLSSPVTKSFNRGEC

SEQ ID NO: 24 - DNA, 318 bp, synthetic construct
  source 1..318: mol_type = other DNA; note = 7G1 CL
actgtcgcagctccatccgtgttcatctttccaccctccgacgagcaactgaaaagtggcacagcctccgtcgtctgtctgctgaacaatttctaccctcgggaggccaaggtccagtggaaggtggacaacgctctccagagtggaaatagccaagagtccgttactgagcaggactctaaggattcaacctacatgctcattagcattctgactctgagcaaggcagattatgagaagcacaaagtctacgcatgtgaagtgactcatcagggactcagctcacccgttaccaagtctttcaacaggggagagtgt

SEQ ID NO: 25 - protein, 98 aa, synthetic construct
  source 1..98: note = 7H11 CH1
ASTKGPSVFPLAPSSKSTSGGTAALGCLVKDYFPEPVTVSWNSGALTSGVHTFPAVLQSSGLYDLYSVVTVPSSSLGTQTYICNVNHKPSNTKVDKKV

SEQ ID NO: 26 - DNA, 294 bp, synthetic construct
  source 1..294: mol_type = other DNA; note = 7H11 CH1
gctagcaccaagggcccatcggtcttccccctggcaccctcctccaagagcacctctgggggcacagcggccctgggctgcctggtcaaggactacttccccgaaccggtgacggtgtcgtggaactcaggcgccctgaccagcggcgtgcacaccttcccggctgtcctacagtcctcaggactctacgatctctatagcgttgtgaccgtgccctccagcagcttgggcacccagacctacatctgcaacgtgaatcacaagcccagcaacaccaaggtggacaagaaagtt

SEQ ID NO: 27 - protein, 106 aa, synthetic construct
  source 1..106: note = 7H11 CL
TVAAPSVFIFPPSDEQLKSGTASVVCLLNNFYPREAKVQWKVDNALQSGNSQESVTEQDSKDSTYNLLSALTLSKADYEKHKVYACEVTHQGLSSPVTKSFNRGEC

SEQ ID NO: 28 - DNA, 318 bp, synthetic construct
  source 1..318: mol_type = other DNA; note = 7H11 CL
actgtcgcagctccatccgtgttcatctttccaccctccgacgagcaactgaaaagtggcacagcctccgtcgtctgtctgctgaacaatttctaccctcgggaggccaaggtccagtggaaggtggacaacgctctccagagtggaaatagccaagagtccgttactgagcaggactctaaggattcaacctacaatctcctgagcgcgctgactctgagcaaggcagattatgagaagcacaaagtctacgcatgtgaagtgactcatcagggactcagctcacccgttaccaagtctttcaacaggggagagtgt

SEQ ID NO: 29 - protein, 98 aa, synthetic construct
  source 1..98: note = 8C10 CH1
ASTKGPSVFPLAPSSKSTSGGTAALGCLVKDYFPEPVTVSWNSGALTSGVHTFPAVLQSSGLYKLVSYVTVPSSSLGTQTYICNVNHKPSNTKVDKKV

SEQ ID NO: 30 - DNA, 294 bp, synthetic construct
  source 1..294: mol_type = other DNA; note = 8C10 CH1
gctagcaccaagggcccatcggtcttccccctggcaccctcctccaagagcacctctgggggcacagcggccctgggctgcctggtcaaggactacttccccgaaccggtgacggtgtcgtggaactcaggcgccctgaccagcggcgtgcacaccttcccggctgtcctacagtcctcaggactctacaagctcgtgagctatgtgaccgtgccctccagcagcttgggcacccagacctacatctgcaacgtgaatcacaagcccagcaacaccaaggtggacaagaaagtt

SEQ ID NO: 31 - protein, 106 aa, synthetic construct
  source 1..106: note = 8C10 CL
TVAAPSVFIFPPSDEQLKSGTASVVCLLNNFYPREAKVQWKVDNALQSGNSQESVTEQDSKDSTYNLYSLLTLSKADYEKHKVYACEVTHQGLSSPVTKSFNRGEC

SEQ ID NO: 32 - DNA, 318 bp, synthetic construct
  source 1..318: mol_type = other DNA; note = 8C10 CL
actgtcgcagctccatccgtgttcatctttccaccctccgacgagcaactgaaaagtggcacagcctccgtcgtctgtctgctgaacaatttctaccctcgggaggccaaggtccagtggaaggtggacaacgctctccagagtggaaatagccaagagtccgttactgagcaggactctaaggattcaacctacaatctctatagcctgctgactctgagcaaggcagattatgagaagcacaaagtctacgcatgtgaagtgactcatcagggactcagctcacccgttaccaagtctttcaacaggggagagtgt

SEQ ID NO: 33 - protein, 98 aa, synthetic construct
  source 1..98: note = 8D6 CH1
ASTKGPSVFPLAPSSKSTSGGTAALGCLVKDYFPEPVTVSWNSGALTSGVHTFPAVLQSSGLYTLYSFVTVPSSSLGTQTYICNVNHKPSNTKVDKKV

SEQ ID NO: 34 - DNA, 294 bp, synthetic construct
  source 1..294: mol_type = other DNA; note = 8D6 CH1
gctagcaccaagggcccatcggtcttccccctggcaccctcctccaagagcacctctgggggcacagcggccctgggctgcctggtcaaggactacttccccgaaccggtgacggtgtcgtggaactcaggcgccctgaccagcggcgtgcacaccttcccggctgtcctacagtcctcaggactctacacgctctatagctttgtgaccgtgccctccagcagcttgggcacccagacctacatctgcaacgtgaatcacaagcccagcaacaccaaggtggacaagaaagtt

SEQ ID NO: 35 - protein, 106 aa, synthetic construct
  source 1..106: note = 8D6 CL
TVAAPSVFIFPPSDEQLKSGTASVVCLLNNFYPREAKVQWKVDNALQSGNSQESVTEQDSKDSTYALESALTLSKADYEKHKVYACEVTHQGLSSPVTKSFNRGEC

SEQ ID NO: 36 - DNA, 318 bp, synthetic construct
  source 1..318: mol_type = other DNA; note = 8D6 CL
actgtcgcagctccatccgtgttcatctttccaccctccgacgagcaactgaaaagtggcacagcctccgtcgtctgtctgctgaacaatttctaccctcgggaggccaaggtccagtggaaggtggacaacgctctccagagtggaaatagccaagagtccgttactgagcaggactctaaggattcaacctacgctctcgagagcgctctgactctgagcaaggcagattatgagaagcacaaagtctacgcatgtgaagtgactcatcagggactcagctcacccgttaccaagtctttcaacaggggagagtgt

SEQ ID NO: 37 - protein, 98 aa, synthetic construct
  source 1..98: note = 8E10 CH1
ASTKGPSVFPLAPSSKSTSGGTAALGCLVKDYFPEPVTVSWNSGALTSGVHTFPAVLQSSGLYMLLSVVTVPSSSLGTQTYICNVNHKPSNTKVDKKV

SEQ ID NO: 38 - DNA, 294 bp, synthetic construct
  source 1..294: mol_type = other DNA; note = 8E10 CH1
gctagcaccaagggcccatcggtcttccccctggcaccctcctccaagagcacctctgggggcacagcggccctgggctgcctggtcaaggactacttccccgaaccggtgacggtgtcgtggaactcaggcgccctgaccagcggcgtgcacaccttcccggctgtcctacagtcctcaggactctacatgctcttgagcgttgtgaccgtgccctccagcagcttgggcacccagacctacatctgcaacgtgaatcacaagcccagcaacaccaaggtggacaagaaagtt

SEQ ID NO: 39 - protein, 106 aa, synthetic construct
  source 1..106: note = 8E10 CL
TVAAPSVFIFPPSDEQLKSGTASVVCLLNNFYPREAKVQWKVDNALQSGNSQESVTEQDSKDSTYTLASVLTLSKADYEKHKVYACEVTHQGLSSPVTKSFNRGEC

SEQ ID NO: 40 - DNA, 318 bp, synthetic construct
  source 1..318: mol_type = other DNA; note = 8E10 CL
actgtcgcagctccatccgtgttcatctttccaccctccgacgagcaactgaaaagtggcacagcctccgtcgtctgtctgctgaacaatttctaccctcgggaggccaaggtccagtggaaggtggacaacgctctccagagtggaaatagccaagagtccgttactgagcaggactctaaggattcaacctacacgctcgctagcgttctgactctgagcaaggcagattatgagaagcacaaagtctacgcatgtgaagtgactcatcagggactcagctcacccgttaccaagtctttcaacaggggagagtgt

SEQ ID NO: 41 - protein, 98 aa, synthetic construct
  source 1..98: note = 8F11 CH1
ASTKGPSVFPLAPSSKSTSGGTAALGCLVKDYFPEPVTVSWNSGALTSGVHTFPAVLQSSGLYTLFSLVTVPSSSLGTQTYICNVNHKPSNTKVDKKV

SEQ ID NO: 42 - DNA, 294 bp, synthetic construct
  source 1..294: mol_type = other DNA; note = 8F11 CH1
gctagcaccaagggcccatcggtcttccccctggcaccctcctccaagagcacctctgggggcacagcggccctgggctgcctggtcaaggactacttccccgaaccggtgacggtgtcgtggaactcaggcgccctgaccagcggcgtgcacaccttcccggctgtcctacagtcctcaggactctacactctctttagccttgtgaccgtgccctccagcagcttgggcacccagacctacatctgcaacgtgaatcacaagcccagcaacaccaaggtggacaagaaagtt

SEQ ID NO: 43 - protein, 106 aa, synthetic construct
  source 1..106: note = 8F11 CL
TVAAPSVFIFPPSDEQLKSGTASVVCLLNNFYPREAKVQWKVDNALQSGNSQESVTEQDSKDSTYWLTSLLTLSKADYEKHKVYACEVTHQGLSSPVTKSFNRGEC

SEQ ID NO: 44 - DNA, 318 bp, synthetic construct
  source 1..318: mol_type = other DNA; note = 8F11 CL
actgtcgcagctccatccgtgttcatctttccaccctccgacgagcaactgaaaagtggcacagcctccgtcgtctgtctgctgaacaatttctaccctcgggaggccaaggtccagtggaaggtggacaacgctctccagagtggaaatagccaagagtccgttactgagcaggactctaaggattcaacctactggctcacgagcttgctgactctgagcaaggcagattatgagaagcacaaagtctacgcatgtgaagtgactcatcagggactcagctcacccgttaccaagtctttcaacaggggagagtgt

SEQ ID NO: 45 - protein, 98 aa, synthetic construct
  source 1..98: note = 8G5 CH1
ASTKGPSVFPLAPSSKSTSGGTAALGCLVKDYFPEPVTVSWNSGALTSGVHTFPAVLQSSGLYVLISQVTVPSSSLGTQTYICNVNHKPSNTKVDKKV

SEQ ID NO: 46 - DNA, 294 bp, synthetic construct
  source 1..294: mol_type = other DNA; note = 8G5 CH1
gctagcaccaagggcccatcggtcttccccctggcaccctcctccaagagcacctctgggggcacagcggccctgggctgcctggtcaaggactacttccccgaaccggtgacggtgtcgtggaactcaggcgccctgaccagcggcgtgcacaccttcccggctgtcctacagtcctcaggactctacgttctcattagccaggtgaccgtgccctccagcagcttgggcacccagacctacatctgcaacgtgaatcacaagcccagcaacaccaaggtggacaagaaagtt

SEQ ID NO: 47 - protein, 106 aa, synthetic construct
  source 1..106: note = 8G5 CL
TVAAPSVFIFPPSDEQLKSGTASVVCLLNNFYPREAKVQWKVDNALQSGNSQESVTEQDSKDSTYSLASILTLSKADYEKHKVYACEVTHQGLSSPVTKSFNRGEC

SEQ ID NO: 48 - DNA, 318 bp, synthetic construct
  source 1..318: mol_type = other DNA; note = 8G5 CL
actgtcgcagctccatccgtgttcatctttccaccctccgacgagcaactgaaaagtggcacagcctccgtcgtctgtctgctgaacaatttctaccctcgggaggccaaggtccagtggaaggtggacaacgctctccagagtggaaatagccaagagtccgttactgagcaggactctaaggattcaacctactctctcgcgagcattctgactctgagcaaggcagattatgagaagcacaaagtctacgcatgtgaagtgactcatcagggactcagctcacccgttaccaagtctttcaacaggggagagtgt

SEQ ID NO: 49 - protein, 98 aa, synthetic construct
  source 1..98: note = 8H5 CH1
ASTKGPSVFPLAPSSKSTSGGTAALGCLVKDYFPEPVTVSWNSGALTSGVHTFPAVLQSSGLYSLVSYVTVPSSSLGTQTYICNVNHKPSNTKVDKKV

SEQ ID NO: 50 - DNA, 294 bp, synthetic construct
  source 1..294: mol_type = other DNA; note = 8H5 CH1
gctagcaccaagggcccatcggtcttccccctggcaccctcctccaagagcacctctgggggcacagcggccctgggctgcctggtcaaggactacttccccgaaccggtgacggtgtcgtggaactcaggcgccctgaccagcggcgtgcacaccttcccggctgtcctacagtcctcaggactctactcgctcgtgagctatgtgaccgtgccctccagcagcttgggcacccagacctacatctgcaacgtgaatcacaagcccagcaacaccaaggtggacaagaaagtt

SEQ ID NO: 51 - protein, 106 aa, synthetic construct
  source 1..106: note = 8H5 CL
TVAAPSVFIFPPSDEQLKSGTASVVCLLNNFYPREAKVQWKVDNALQSGNSQESVTEQDSKDSTYTLYSSLTLSKADYEKHKVYACEVTHQGLSSPVTKSFNRGEC

SEQ ID NO: 52 - DNA, 318 bp, synthetic construct
  source 1..318: mol_type = other DNA; note = 8H5 CL
actgtcgcagctccatccgtgttcatctttccaccctccgacgagcaactgaaaagtggcacagcctccgtcgtctgtctgctgaacaatttctaccctcgggaggccaaggtccagtggaaggtggacaacgctctccagagtggaaatagccaagagtccgttactgagcaggactctaaggattcaacctacactctctatagctcgctgactctgagcaaggcagattatgagaagcacaaagtctacgcatgtgaagtgactcatcagggactcagctcacccgttaccaagtctttcaacaggggagagtgt

SEQ ID NO: 53 - protein, 98 aa, synthetic construct
  source 1..98: note = 11B7 CH1
ASTKGPSVFPLAPSSKSTSGGTAALGCLVKDYFPEPVTVSWNSGALTSGVHTFPAVLQSSGLYVLLSMVTVPSSSLGTQTYICNVNHKPSNTKVDKKV

SEQ ID NO: 54 - DNA, 294 bp, synthetic construct
  source 1..294: mol_type = other DNA; note = 11B7 CH1
gctagcaccaagggcccatcggtcttccccctggcaccctcctccaagagcacctctgggggcacagcggccctgggctgcctggtcaaggactacttccccgaaccggtgacggtgtcgtggaactcaggcgccctgaccagcggcgtgcacaccttcccggctgtcctacagtcctcaggactctacgtgctcttgagcatggtgaccgtgccctccagcagcttgggcacccagacctacatctgcaacgtgaatcacaagcccagcaacaccaaggtggacaagaaagtt

SEQ ID NO: 55 - protein, 106 aa, synthetic construct
  source 1..106: note = 11B7 CL
TVAAPSVFIFPPSDEQLKSGTASVVCLLNNFYPREAKVQWKVDNALQSGNSQESVTEQDSKDSTYRLWSLLTLSKADYEKHKVYACEVTHQGLSSPVTKSFNRGEC

SEQ ID NO: 56 - DNA, 318 bp, synthetic construct
  source 1..318: mol_type = other DNA; note = 11B7 CL
actgtcgcagctccatccgtgttcatctttccaccctccgacgagcaactgaaaagtggcacagcctccgtcgtctgtctgctgaacaatttctaccctcgggaggccaaggtccagtggaaggtggacaacgctctccagagtggaaatagccaagagtccgttactgagcaggactctaaggattcaacctaccgtctctggagccttctgactctgagcaaggcagattatgagaagcacaaagtctacgcatgtgaagtgactcatcagggactcagctcacccgttaccaagtctttcaacaggggagagtgt

SEQ ID NO: 57 - protein, 98 aa, synthetic construct
  source 1..98: note = 11C8 CH1
ASTKGPSVFPLAPSSKSTSGGTAALGCLVKDYFPEPVTVSWNSGALTSGVHTFPAVLQSSGLYMLVSTVTVPSSSLGTQTYICNVNHKPSNTKVDKKV

SEQ ID NO: 58 - DNA, 294 bp, synthetic construct
  source 1..294: mol_type = other DNA; note = 11C8 CH1
gctagcaccaagggcccatcggtcttccccctggcaccctcctccaagagcacctctgggggcacagcggccctgggctgcctggtcaaggactacttccccgaaccggtgacggtgtcgtggaactcaggcgccctgaccagcggcgtgcacaccttcccggctgtcctacagtcctcaggactctacatgctcgttagcacggtgaccgtgccctccagcagcttgggcacccagacctacatctgcaacgtgaatcacaagcccagcaacaccaaggtggacaagaaagtt

SEQ ID NO: 59 - protein, 106 aa, synthetic construct
  source 1..106: note = 11C8 CL
TVAAPSVFIFPPSDEQLKSGTASVVCLLNNFYPREAKVQWKVDNALQSGNSQESVTEQDSKDSTYSLTNYLTLSKADYEKHKVYACEVTHQGLSSPVTKSFNRGEC

SEQ ID NO: 60 - DNA, 318 bp, synthetic construct
  source 1..318: mol_type = other DNA; note = 11C8 CL
actgtcgcagctccatccgtgttcatctttccaccctccgacgagcaactgaaaagtggcacagcctccgtcgtctgtctgctgaacaatttctaccctcgggaggccaaggtccagtggaaggtggacaacgctctccagagtggaaatagccaagagtccgttactgagcaggactctaaggattcaacctacagtctcactaactatctgactctgagcaaggcagattatgagaagcacaaagtctacgcatgtgaagtgactcatcagggactcagctcacccgttaccaagtctttcaacaggggagagtgt

SEQ ID NO: 61 - protein, 98 aa, synthetic construct
  source 1..98: note = 11F5 CH1
ASTKGPSVFPLAPSSKSTSGGTAALGCLVKDYFPEPVTVSWNSGALTSGVHTFPAVLQSSGLYALFSSVTVPSSSLGTQTYICNVNHKPSNTKVDKKV

SEQ ID NO: 62 - DNA, 294 bp, synthetic construct
  source 1..294: mol_type = other DNA; note = 11F5 CH1
gctagcaccaagggcccatcggtcttccccctggcaccctcctccaagagcacctctgggggcacagcggccctgggctgcctggtcaaggactacttccccgaaccggtgacggtgtcgtggaactcaggcgccctgaccagcggcgtgcacaccttcccggctgtcctacagtcctcaggactctacgctctctttagctctgtgaccgtgccctccagcagcttgggcacccagacctacatctgcaacgtgaatcacaagcccagcaacaccaaggtggacaagaaagtt

SEQ ID NO: 63 - protein, 106 aa, synthetic construct
  source 1..106: note = 11F5 CL
TVAAPSVFIFPPSDEQLKSGTASVVCLLNNFYPREAKVQWKVDNALQSGNSQESVTEQDSKDSTYSLYSVLTLSKADYEKHKVYACEVTHQGLSSPVTKSFNRGEC

SEQ ID NO: 64 - DNA, 318 bp, synthetic construct
  source 1..318: mol_type = other DNA; note = 11F5 CL
actgtcgcagctccatccgtgttcatctttccaccctccgacgagcaactgaaaagtggcacagcctccgtcgtctgtctgctgaacaatttctaccctcgggaggccaaggtccagtggaaggtggacaacgctctccagagtggaaatagccaagagtccgttactgagcaggactctaaggattcaacctacagtctctatagcgtgctgactctgagcaaggcagattatgagaagcacaaagtctacgcatgtgaagtgactcatcagggactcagctcacccgttaccaagtctttcaacaggggagagtgt

SEQ ID NO: 65 - protein, 98 aa, synthetic construct
  source 1..98: note = 11H7 CH1
ASTKGPSVFPLAPSSKSTSGGTAALGCLVKDYFPEPVTVSWNSGALTSGVHTFPAVLQSSGLYELLSIVTVPSSSLGTQTYICNVNHKPSNTKVDKKV

SEQ ID NO: 66 - DNA, 294 bp, synthetic construct
  source 1..294: mol_type = other DNA; note = 11H7 CH1
gctagcaccaagggcccatcggtcttccccctggcaccctcctccaagagcacctctgggggcacagcggccctgggctgcctggtcaaggactacttccccgaaccggtgacggtgtcgtggaactcaggcgccctgaccagcggcgtgcacaccttcccggctgtcctacagtcctcaggactctacgagctccttagcattgtgaccgtgccctccagcagcttgggcacccagacctacatctgcaacgtgaatcacaagcccagcaacaccaaggtggacaagaaagtt

SEQ ID NO: 67 - protein, 106 aa, synthetic construct
  source 1..106: note = 11H7 CL
TVAAPSVFIFPPSDEQLKSGTASVVCLLNNFYPREAKVQWKVDNALQSGNSQESVTEQDSKDSTYNLSSLLTLSKADYEKHKVYACEVTHQGLSSPVTKSFNRGEC

SEQ ID NO: 68 - DNA, 318 bp, synthetic construct
  source 1..318: mol_type = other DNA; note = 11H7 CL
actgtcgcagctccatccgtgttcatctttccaccctccgacgagcaactgaaaagtggcacagcctccgtcgtctgtctgctgaacaatttctaccctcgggaggccaaggtccagtggaaggtggacaacgctctccagagtggaaatagccaagagtccgttactgagcaggactctaaggattcaacctacaatctctctagcctgctgactctgagcaaggcagattatgagaagcacaaagtctacgcatgtgaagtgactcatcagggactcagctcacccgttaccaagtctttcaacaggggagagtgt

SEQ ID NO: 69 - protein, 98 aa, synthetic construct
  source 1..98: note = 12B2 CH1
ASTKGPSVFPLAPSSKSTSGGTAALGCLVKDYFPEPVTVSWNSGALTSGVHTFPAVLQSSGLYTLVSFVTVPSSSLGTQTYICNVNHKPSNTKVDKKV

SEQ ID NO: 70 - DNA, 294 bp, synthetic construct
  source 1..294: mol_type = other DNA; note = 12B2 CH1
gctagcaccaagggcccatcggtcttccccctggcaccctcctccaagagcacctctgggggcacagcggccctgggctgcctggtcaaggactacttccccgaaccggtgacggtgtcgtggaactcaggcgccctgaccagcggcgtgcacaccttcccggctgtcctacagtcctcaggactctacacgctcgttagctttgtgaccgtgccctccagcagcttgggcacccagacctacatctgcaacgtgaatcacaagcccagcaacaccaaggtggacaagaaagtt

SEQ ID NO: 71 - protein, 106 aa, synthetic construct
  source 1..106: note = 12B2 CL
TVAAPSVFIFPPSDEQLKSGTASVVCLLNNFYPREAKVQWKVDNALQSGNSQESVTEQDSKDSTYCLTSVLTLSKADYEKHKVYACEVTHQGLSSPVTKSFNRGEC

SEQ ID NO: 72 - DNA, 318 bp, synthetic construct
  source 1..318: mol_type = other DNA; note = 12B2 CL
actgtcgcagctccatccgtgttcatctttccaccctccgacgagcaactgaaaagtggcacagcctccgtcgtctgtctgctgaacaatttctaccctcgggaggccaaggtccagtggaaggtggacaacgctctccagagtggaaatagccaagagtccgttactgagcaggactctaaggattcaacctactgtctcactagcgttctgactctgagcaaggcagattatgagaagcacaaagtctacgcatgtgaagtgactcatcagggactcagctcacccgttaccaagtctttcaacaggggagagtgt

SEQ ID NO: 73 - protein, 98 aa, synthetic construct
  source 1..98: note = 12D6 CH1
ASTKGPSVFPLAPSSKSTSGGTAALGCLVKDYFPEPVTVSWNSGALTSGVHTFPAVLQSSGLYSLLSIVTVPSSSLGTQTYICNVNHKPSNTKVDKKV

SEQ ID NO: 74 - DNA, 294 bp, synthetic construct
  source 1..294: mol_type = other DNA; note = 12D6 CH1
gctagcaccaagggcccatcggtcttccccctggcaccctcctccaagagcacctctgggggcacagcggccctgggctgcctggtcaaggactacttccccgaaccggtgacggtgtcgtggaactcaggcgccctgaccagcggcgtgcacaccttcccggctgtcctacagtcctcaggactctactctctccttagcattgtgaccgtgccctccagcagcttgggcacccagacctacatctgcaacgtgaatcacaagcccagcaacaccaaggtggacaagaaagtt

SEQ ID NO: 75 - protein, 106 aa, synthetic construct
  source 1..106: note = 12D6 CL
TVAAPSVFIFPPSDEQLKSGTASVVCLLNNFYPREAKVQWKVDNALQSGNSQESVTEQDSKDSTYFLSSLLTLSKADYEKHKVYACEVTHQGLSSPVTKSFNRGEC

SEQ ID NO: 76 - DNA, 318 bp, synthetic construct
  source 1..318: mol_type = other DNA; note = 12D6 CL
actgtcgcagctccatccgtgttcatctttccaccctccgacgagcaactgaaaagtggcacagcctccgtcgtctgtctgctgaacaatttctaccctcgggaggccaaggtccagtggaaggtggacaacgctctccagagtggaaatagccaagagtccgttactgagcaggactctaaggattcaacctactttctctctagcttgctgactctgagcaaggcagattatgagaagcacaaagtctacgcatgtgaagtgactcatcagggactcagctcacccgttaccaagtctttcaacaggggagagtgt

SEQ ID NO: 77 - protein, 98 aa, synthetic construct
  source 1..98: note = 11A10 CH1
ASTKGPSVFPLAPSSKSTSGGTAALGCLVKDYFPEPVTVSWNSGALTSGVHTFPAVLQSSGLYMLISWVTVPSSSLGTQTYICNVNHKPSNTKVDKKV

SEQ ID NO: 78 - DNA, 294 bp, synthetic construct
  source 1..294: mol_type = other DNA; note = 11A10 CH1
gctagcaccaagggcccatcggtcttccccctggcaccctcctccaagagcacctctgggggcacagcggccctgggctgcctggtcaaggactacttccccgaaccggtgacggtgtcgtggaactcaggcgccctgaccagcggcgtgcacaccttcccggctgtcctacagtcctcaggactctacatgctcattagctgggtgaccgtgccctccagcagcttgggcacccagacctacatctgcaacgtgaatcacaagcccagcaacaccaaggtggacaagaaagtt

SEQ ID NO: 79 - protein, 106 aa, synthetic construct
  source 1..106: note = 11A10 CL
TVAAPSVFIFPPSDEQLKSGTASVVCLLNNFYPREAKVQWKVDNALQSGNSQESVTEQDSKDSTYRLHSVLTLSKADYEKHKVYACEVTHQGLSSPVTKSFNRGEC

SEQ ID NO: 80 - DNA, 318 bp, synthetic construct
  source 1..318: mol_type = other DNA; note = 11A10 CL
actgtcgcagctccatccgtgttcatctttccaccctccgacgagcaactgaaaagtggcacagcctccgtcgtctgtctgctgaacaatttctaccctcgggaggccaaggtccagtggaaggtggacaacgctctccagagtggaaatagccaagagtccgttactgagcaggactctaaggattcaacctacaggctccatagcgttctgactctgagcaaggcagattatgagaagcacaaagtctacgcatgtgaagtgactcatcagggactcagctcacccgttaccaagtctttcaacaggggagagtgt

SEQ ID NO: 81 - protein, 98 aa, synthetic construct
  source 1..98: note = 11D6 CH1
ASTKGPSVFPLAPSSKSTSGGTAALGCLVKDYFPEPVTVSWNSGALTSGVHTFPAVLQSSGLYWLFSTVTVPSSSLGTQTYICNVNHKPSNTKVDKKV

SEQ ID NO: 82 - DNA, 294 bp, synthetic construct
  source 1..294: mol_type = other DNA; note = 11D6 CH1
gctagcaccaagggcccatcggtcttccccctggcaccctcctccaagagcacctctgggggcacagcggccctgggctgcctggtcaaggactacttccccgaaccggtgacggtgtcgtggaactcaggcgccctgaccagcggcgtgcacaccttcccggctgtcctacagtcctcaggactctactggctctttagcacggtgaccgtgccctccagcagcttgggcacccagacctacatctgcaacgtgaatcacaagcccagcaacaccaaggtggacaagaaagtt

SEQ ID NO: 83 - protein, 106 aa, synthetic construct
  source 1..106: note = 11D6 CL
TVAAPSVFIFPPSDEQLKSGTASVVCLLNNFYPREAKVQWKVDNALQSGNSQESVTEQDSKDSTYKLVSMLTLSKADYEKHKVYACEVTHQGLSSPVTKSFNRGEC

SEQ ID NO: 84 - DNA, 318 bp, synthetic construct
  source 1..318: mol_type = other DNA; note = 11D6 CL
actgtcgcagctccatccgtgttcatctttccaccctccgacgagcaactgaaaagtggcacagcctccgtcgtctgtctgctgaacaatttctaccctcgggaggccaaggtccagtggaaggtggacaacgctctccagagtggaaatagccaagagtccgttactgagcaggactctaaggattcaacctacaagctcgttagcatgctgactctgagcaaggcagattatgagaagcacaaagtctacgcatgtgaagtgactcatcagggactcagctcacccgttaccaagtctttcaacaggggagagtgt

SEQ ID NO: 85 - protein, 98 aa, synthetic construct
  source 1..98: note = 11C3 CH1
ASTKGPSVFPLAPSSKSTSGGTAALGCLVKDYFPEPVTVSWNSGALTSGVHTFPAVLQSSGLYTLFSSVTVPSSSLGTQTYICNVNHKPSNTKVDKKV

SEQ ID NO: 86 - DNA, 294 bp, synthetic construct
  source 1..294: mol_type = other DNA; note = 11C3 CH1
gctagcaccaagggcccatcggtcttccccctggcaccctcctccaagagcacctctgggggcacagcggccctgggctgcctggtcaaggactacttccccgaaccggtgacggtgtcgtggaactcaggcgccctgaccagcggcgtgcacaccttcccggctgtcctacagtcctcaggactctacacgctctttagctcggtgaccgtgccctccagcagcttgggcacccagacctacatctgcaacgtgaatcacaagcccagcaacaccaaggtggacaagaaagtt

SEQ ID NO: 87 - protein, 106 aa, synthetic construct
  source 1..106: note = 11C3 CL
TVAAPSVFIFPPSDEQLKSGTASVVCLLNNFYPREAKVQWKVDNALQSGNSQESVTEQDSKDSTYHLVSRLTLSKADYEKHKVYACEVTHQGLSSPVTKSFNRGEC

SEQ ID NO: 88 - DNA, 318 bp, synthetic construct
  source 1..318: mol_type = other DNA; note = 11C3 CL
actgtcgcagctccatccgtgttcatctttccaccctccgacgagcaactgaaaagtggcacagcctccgtcgtctgtctgctgaacaatttctaccctcgggaggccaaggtccagtggaaggtggacaacgctctccagagtggaaatagccaagagtccgttactgagcaggactctaaggattcaacctaccatctcgtgagccggctgactctgagcaaggcagattatgagaagcacaaagtctacgcatgtgaagtgactcatcagggactcagctcacccgttaccaagtctttcaacaggggagagtgt

SEQ ID NO: 89 - protein, 98 aa, synthetic construct
  source 1..98: note = 11C12 CH1
ASTKGPSVFPLAPSSKSTSGGTAALGCLVKDYFPEPVTVSWNSGALTSGVHTFPAVLQSSGLYKLLSVVTVPSSSLGTQTYICNVNHKPSNTKVDKKV

SEQ ID NO: 90 - DNA, 294 bp, synthetic construct
  source 1..294: mol_type = other DNA; note = 11C12 CH1
gctagcaccaagggcccatcggtcttccccctggcaccctcctccaagagcacctctgggggcacagcggccctgggctgcctggtcaaggactacttccccgaaccggtgacggtgtcgtggaactcaggcgccctgaccagcggcgtgcacaccttcccggctgtcctacagtcctcaggactctacaagctccttagcgttgtgaccgtgccctccagcagcttgggcacccagacctacatctgcaacgtgaatcacaagcccagcaacaccaaggtggacaagaaagtt

SEQ ID NO: 91 - protein, 106 aa, synthetic construct
  source 1..106: note = 11C12 CL
TVAAPSVFIFPPSDEQLKSGTASVVCLLNNFYPREAKVQWKVDNALQSGNSQESVTEQDSKDSTYYLMSELTLSKADYEKHKVYACEVTHQGLSSPVTKSFNRGEC

SEQ ID NO: 92 - DNA, 318 bp, synthetic construct
  source 1..318: mol_type = other DNA; note = 11C12 CL
actgtcgcagctccatccgtgttcatctttccaccctccgacgagcaactgaaaagtggcacagcctccgtcgtctgtctgctgaacaatttctaccctcgggaggccaaggtccagtggaaggtggacaacgctctccagagtggaaatagccaagagtccgttactgagcaggactctaaggattcaacctactatctcatgagcgagctgactctgagcaaggcagattatgagaagcacaaagtctacgcatgtgaagtgactcatcagggactcagctcacccgttaccaagtctttcaacaggggagagtgt

SEQ ID NO: 93 - protein, 98 aa, synthetic construct
  source 1..98: note = 11F6 CH1
ASTKGPSVFPLAPSSKSTSGGTAALGCLVKDYFPEPVTVSWNSGALTSGVHTFPAVLQSSGLYALISIVTVPSSSLGTQTYICNVNHKPSNTKVDKKV

SEQ ID NO: 94 - DNA, 294 bp, synthetic construct
  source 1..294: mol_type = other DNA; note = 11F6 CH1
gctagcaccaagggcccatcggtcttccccctggcaccctcctccaagagcacctctgggggcacagcggccctgggctgcctggtcaaggactacttccccgaaccggtgacggtgtcgtggaactcaggcgccctgaccagcggcgtgcacaccttcccggctgtcctacagtcctcaggactctacgcgctcattagcattgtgaccgtgccctccagcagcttgggcacccagacctacatctgcaacgtgaatcacaagcccagcaacaccaaggtggacaagaaagtt

SEQ ID NO: 95 - protein, 106 aa, synthetic construct
  source 1..106: note = 11F6 CL
TVAAPSVFIFPPSDEQLKSGTASVVCLLNNFYPREAKVQWKVDNALQSGNSQESVTEQDSKDSTYNLESMLTLSKADYEKHKVYACEVTHQGLSSPVTKSFNRGEC

SEQ ID NO: 96 - DNA, 318 bp, synthetic construct
  source 1..318: mol_type = other DNA; note = 11F6 CL
actgtcgcagctccatccgtgttcatctttccaccctccgacgagcaactgaaaagtggcacagcctccgtcgtctgtctgctgaacaatttctaccctcgggaggccaaggtccagtggaaggtggacaacgctctccagagtggaaatagccaagagtccgttactgagcaggactctaaggattcaacctacaatctcgagagcatgctgactctgagcaaggcagattatgagaagcacaaagtctacgcatgtgaagtgactcatcagggactcagctcacccgttaccaagtctttcaacaggggagagtgt

SEQ ID NO: 97 - protein, 98 aa, synthetic construct
  source 1..98: note = 11F8 CH1
ASTKGPSVFPLAPSSKSTSGGTAALGCLVKDYFPEPVTVSWNSGALTSGVHTFPAVLQSSGLYSLVSIVTVPSSSLGTQTYICNVNHKPSNTKVDKKV

SEQ ID NO: 98 - DNA, 294 bp, synthetic construct
  source 1..294: mol_type = other DNA; note = 11F8 CH1
gctagcaccaagggcccatcggtcttccccctggcaccctcctccaagagcacctctgggggcacagcggccctgggctgcctggtcaaggactacttccccgaaccggtgacggtgtcgtggaactcaggcgccctgaccagcggcgtgcacaccttcccggctgtcctacagtcctcaggactctacagtctcgtgagcattgtgaccgtgccctccagcagcttgggcacccagacctacatctgcaacgtgaatcacaagcccagcaacaccaaggtggacaagaaagtt

SEQ ID NO: 99 - protein, 106 aa, synthetic construct
  source 1..106: note = 11F8 CL
TVAAPSVFIFPPSDEQLKSGTASVVCLLNNFYPREAKVQWKVDNALQSGNSQESVTEQDSKDSTYFLLSSLTLSKADYEKHKVYACEVTHQGLSSPVTKSFNRGEC

SEQ ID NO: 100 - DNA, 318 bp, synthetic construct
  source 1..318: mol_type = other DNA; note = 11F8 CL
actgtcgcagctccatccgtgttcatctttccaccctccgacgagcaactgaaaagtggcacagcctccgtcgtctgtctgctgaacaatttctaccctcgggaggccaaggtccagtggaaggtggacaacgctctccagagtggaaatagccaagagtccgttactgagcaggactctaaggattcaacctactttctcttgagctcgctgactctgagcaaggcagattatgagaagcacaaagtctacgcatgtgaagtgactcatcagggactcagctcacccgttaccaagtctttcaacaggggagagtgt

SEQ ID NO: 101 - protein, 98 aa, synthetic construct
  source 1..98: note = 11H5 CH1
ASTKGPSVFPLAPSSKSTSGGTAALGCLVKDYFPEPVTVSWNSGALTSGVHTFPAVLQSSGLYTLTSLVTVPSSSLGTQTYICNVNHKPSNTKVDKKV

SEQ ID NO: 102 - DNA, 294 bp, synthetic construct
  source 1..294: mol_type = other DNA; note = 11H5 CH1
gctagcaccaagggcccatcggtcttccccctggcaccctcctccaagagcacctctgggggcacagcggccctgggctgcctggtcaaggactacttccccgaaccggtgacggtgtcgtggaactcaggcgccctgaccagcggcgtgcacaccttcccggctgtcctacagtcctcaggactctacacgctcactagcttggtgaccgtgccctccagcagcttgggcacccagacctacatctgcaacgtgaatcacaagcccagcaacaccaaggtggacaagaaagtt

SEQ ID NO: 103 - protein, 106 aa, synthetic construct
  source 1..106: note = 11H5 CL
TVAAPSVFIFPPSDEQLKSGTASVVCLLNNFYPREAKVQWKVDNALQSGNSQESVTEQDSKDSTYYLSSILTLSKADYEKHKVYACEVTHQGLSSPVTKSFNRGEC

SEQ ID NO: 104 - DNA, 318 bp, synthetic construct
  source 1..318: mol_type = other DNA; note = 11H5 CL
actgtcgcagctccatccgtgttcatctttccaccctccgacgagcaactgaaaagtggcacagcctccgtcgtctgtctgctgaacaatttctaccctcgggaggccaaggtccagtggaaggtggacaacgctctccagagtggaaatagccaagagtccgttactgagcaggactctaaggattcaacctactatctcagtagcattctgactctgagcaaggcagattatgagaagcacaaagtctacgcatgtgaagtgactcatcagggactcagctcacccgttaccaagtctttcaacaggggagagtgt

SEQ ID NO: 105 - protein, 98 aa, synthetic construct
  source 1..98: note = 11H2 CH1
ASTKGPSVFPLAPSSKSTSGGTAALGCLVKDYFPEPVTVSWNSGALTSGVHTFPAVLQSSGLYYLMSFVTVPSSSLGTQTYICNVNHKPSNTKVDKKV

SEQ ID NO: 106 - DNA, 294 bp, synthetic construct
  source 1..294: mol_type = other DNA; note = 11H2 CH1
gctagcaccaagggcccatcggtcttccccctggcaccctcctccaagagcacctctgggggcacagcggccctgggctgcctggtcaaggactacttccccgaaccggtgacggtgtcgtggaactcaggcgccctgaccagcggcgtgcacaccttcccggctgtcctacagtcctcaggactctactatctcatgagctttgtgaccgtgccctccagcagcttgggcacccagacctacatctgcaacgtgaatcacaagcccagcaacaccaaggtggacaagaaagtt

SEQ ID NO: 107 - protein, 106 aa, synthetic construct
  source 1..106: note = 11H2 CL
TVAAPSVFIFPPSDEQLKSGTASVVCLLNNFYPREAKVQWKVDNALQSGNSQESVTEQDSKDSTYSLVSTLTLSKADYEKHKVYACEVTHQGLSSPVTKSFNRGEC

SEQ ID NO: 108 - DNA, 318 bp, synthetic construct
  source 1..318: mol_type = other DNA; note = 11H2 CL
actgtcgcagctccatccgtgttcatctttccaccctccgacgagcaactgaaaagtggcacagcctccgtcgtctgtctgctgaacaatttctaccctcgggaggccaaggtccagtggaaggtggacaacgctctccagagtggaaatagccaagagtccgttactgagcaggactctaaggattcaacctactcgctcgtgagcacgctgactctgagcaaggcagattatgagaagcacaaagtctacgcatgtgaagtgactcatcagggactcagctcacccgttaccaagtctttcaacaggggagagtgt

SEQ ID NO: 109 - protein, 98 aa, synthetic construct
  source 1..98: note = 12C3 CH1
ASTKGPSVFPLAPSSKSTSGGTAALGCLVKDYFPEPVTVSWNSGALTSGVHTFPAVLQSSGLYTLMSSVTVPSSSLGTQTYICNVNHKPSNTKVDKKV

SEQ ID NO: 110 - DNA, 294 bp, synthetic construct
  source 1..294: mol_type = other DNA; note = 12C3 CH1
gctagcaccaagggcccatcggtcttccccctggcaccctcctccaagagcacctctgggggcacagcggccctgggctgcctggtcaaggactacttccccgaaccggtgacggtgtcgtggaactcaggcgccctgaccagcggcgtgcacaccttcccggctgtcctacagtcctcaggactctacactctcatgagcagtgtgaccgtgccctccagcagcttgggcacccagacctacatctgcaacgtgaatcacaagcccagcaacaccaaggtggacaagaaagtt

SEQ ID NO: 111 - protein, 106 aa, synthetic construct
  source 1..106: note = 12C3 CL
TVAAPSVFIFPPSDEQLKSGTASVVCLLNNFYPREAKVQWKVDNALQSGNSQESVTEQDSKDSTYLLWSMLTLSKADYEKHKVYACEVTHQGLSSPVTKSFNRGEC

SEQ ID NO: 112 - DNA, 318 bp, synthetic construct
  source 1..318: mol_type = other DNA; note = 12C3 CL
actgtcgcagctccatccgtgttcatctttccaccctccgacgagcaactgaaaagtggcacagcctccgtcgtctgtctgctgaacaatttctaccctcgggaggccaaggtccagtggaaggtggacaacgctctccagagtggaaatagccaagagtccgttactgagcaggactctaaggattcaacctacctgctctggagcatgctgactctgagcaaggcagattatgagaagcacaaagtctacgcatgtgaagtgactcatcagggactcagctcacccgttaccaagtctttcaacaggggagagtgt

SEQ ID NO: 113 - protein, 98 aa, synthetic construct
  source 1..98: note = 7A10 CH1
ASTKGPSVFPLAPSSKSTSGGTAALGCLVKDYFPEPVTVSWNSGALTSGVHTFPAVLQSSGLYTLRSFVTVPSSSLGTQTYICNVNHKPSNTKVDKKV

SEQ ID NO: 114 - DNA, 294 bp, synthetic construct
  source 1..294: mol_type = other DNA; note = 7A10 CH1
gctagcaccaagggcccatcggtcttccccctggcaccctcctccaagagcacctctgggggcacagcggccctgggctgcctggtcaaggactacttccccgaaccggtgacggtgtcgtggaactcaggcgccctgaccagcggcgtgcacaccttcccggctgtcctacagtcctcaggactctacacgctccgtagctttgtgaccgtgccctccagcagcttgggcacccagacctacatctgcaacgtgaatcacaagcccagcaacaccaaggtggacaagaaagtt

SEQ ID NO: 115 - protein, 106 aa, synthetic construct
  source 1..106: note = 7A10 CL
TVAAPSVFIFPPSDEQLKSGTASVVCLLNNFYPREAKVQWKVDNALQSGNSQESVTEQDSKDSTYSLSSVLTLSKADYEKHKVYACEVTHQGLSSPVTKSFNRGEC

SEQ ID NO: 116 - DNA, 318 bp, synthetic construct
  source 1..318: mol_type = other DNA; note = 7A10 CL
actgtcgcagctccatccgtgttcatctttccaccctccgacgagcaactgaaaagtggcacagcctccgtcgtctgtctgctgaacaatttctaccctcgggaggccaaggtccagtggaaggtggacaacgctctccagagtggaaatagccaagagtccgttactgagcaggactctaaggattcaacctacagcctctccagcgtgctgactctgagcaaggcagattatgagaagcacaaagtctacgcatgtgaagtgactcatcagggactcagctcacccgttaccaagtctttcaacaggggagagtgt

SEQ ID NO: 117 - protein, 216 aa, synthetic construct
  source 1..216: note = anti-CD3 light chain; note (original language) = 抗CD3轻链
DIQMTQEPSLTTSPGGTVTLTCRSSTGAVTTSNYANWVQEKPGQAPRGLIGGTNKRAPGTPARFSGSLIGGKAALTITGVQPEDEAIYFCALWYSNLWVFGGGTKLEIKRTVAAPSVFIFPPSDEQLKSGTASVVCLLNNFYPREAKVQWKVDNALQSGNSQESVTEQDSKDSTYSLSSTLTLSKADYEKHKVYACEVTHQGLSSPVTKSFNRGEC

SEQ ID NO: 118 - DNA, 648 bp, synthetic construct
  source 1..648: mol_type = other DNA; note = anti-CD3 light chain; note (original language) = 抗CD3轻链
gatattcagatgacacaagaaccaagtctcactacaagccctggaggcaccgttacactgacctgtcgctcttccactggcgccgtgaccacttccaactatgcaaactgggtgcaggagaaacctggacaggctcctagaggtctgattggaggcactaacaagagagctccagggactcctgccaggttcagcggatctctgatcggtgggaaggcagctctgacaatcactggagtgcaacccgaggatgaggctatctacttctgtgctctctggtactcaaatctgtgggtgttcggaggtggaacaaagctggagatcaagcggactgtcgcagctccatccgtgttcatctttccaccctccgacgagcaactgaaaagtggcacagcctccgtcgtctgtctgctgaacaatttctaccctcgggaggccaaggtccagtggaaggtggacaacgctctccagagtggaaatagccaagagtccgttactgagcaggactctaaggattcaacctacagcctctccagcaccctgactctgagcaaggcagattatgagaagcacaaagtctacgcatgtgaagtgactcatcagggactcagctcacccgttaccaagtctttcaacaggggagagtgt

SEQ ID NO: 119 - protein, 455 aa, synthetic construct
  source 1..455: note = anti-CD3 heavy chain; note (original language) = 抗CD3重链
EVQLVESGGGLVQPGGSLKLSCAASGFTFNTYAMNWVRQAPGKGLEWVARIRSKYNNYATYYADSVKDRFTISRDDSKNTAYLQMNNLKTEDTAMYYCVRHGNFGTSYVSWFAYWGQGTLVTVSSASTKGPSVFPLAPSSKSTSGGTAALGCLVKDYFPEPVTVSWNSGALTSGVHTFPAVLQSSGLYSLSSVVTVPSSSLGTQTYICNVNHKPSNTKVDKKVEPKSCDKTHTCPPCPAPEAAGGPSVFLFPPKPKDTLMISRTPEVTCVVVDVSHEDPEVKFNWYVDGVEVHNAKTKPREEQYNSTYRVVSVLTVLHQDWLNGKEYKCKVSNKALPAPIEKTISKAKGQPREPQVYTLPPSREEMTKNQVSLTCLVKGFYPSDIAVEWESNGQPENNYKTTKKKLDSDGSFFLYSKLTVDKSRWQQGNVFSCSVMHEALHNHYTQKSLSLSPGK

SEQ ID NO: 120 - DNA, 1365 bp, synthetic construct
  source 1..1365: mol_type = other DNA; note = anti-CD3 heavy chain; note (original language) = 抗CD3重链
gaagtgcaactggttgaaagcggtggaggactggttcagcctggaggctccctcaaactcagttgcgccgcttccggttttacattcaacacttatgccatgaattgggtgcgccaggctcccggaaaaggcctggaatgggtggcacggatcaggagcaaatacaacaattacgccacatattacgctgactccgttaaagacagattcacaatttccagagatgattccaagaatactgcttatctccagatgaacaacctgaagacagaggatacagctatgtactattgcgtgcggcatggcaatttcggaaattcctatgtgagttggtttgcctactggggacagggaactctcgttactgtcagctccgctagcaccaagggcccatcggtcttccccctggcaccctcctccaagagcacctctgggggcacagcggccctgggctgcctggtcaaggactacttccccgaaccggtgacggtgtcgtggaactcaggcgccctgaccagcggcgtgcacaccttcccggctgtcctacagtcctcaggactctactccctcagcagcgtggtgaccgtgccctccagcagcttgggcacccagacctacatctgcaacgtgaatcacaagcccagcaacaccaaggtggacaagaaagttgagcccaaatcttgtgacaaaactcacacatgcccaccgtgcccagcacctgaagccgcagggggaccgtcagtcttcctcttccccccaaaacccaaggacaccctcatgatctcccggacccctgaggtcacatgcgtggtggtggacgtgagccacgaagaccctgaggtcaagttcaactggtacgtggacggcgtggaggtgcataatgccaagacaaagccgcgggaggagcagtacaacagcacgtaccgtgtggtcagcgtcctcaccgtcctgcaccaggactggctgaatggcaaggagtacaagtgcaaggtctccaacaaagccctcccagcccccatcgagaaaaccatctccaaagccaaagggcagccccgagaaccacaggtgtacaccctgcccccatcccgggaggagatgaccaagaaccaggtcagcctgacctgcctggtcaaaggcttctatcccagcgacatcgccgtggagtgggagagcaatgggcagccggagaacaactacaagaccacgaagaagaagctggactccgacggctccttcttcctctacagcaagctcaccgtggacaagagcaggtggcagcaggggaacgtcttctcatgctccgtgatgcatgaggctctgcacaaccactacacgcagaagagcctctccctgtctccgggtaaa

SEQ ID NO: 121 - protein, 218 aa, synthetic construct
  source 1..218: note = anti-GPC3 light chain; note (original language) = 抗GPC3轻链
DIVLTQSPLSLTVTPGEPASISCRSSESLVHSNGNTYLSWLQQRPGQPPRLLIYKISNRFSGVPDRFSGSGAGTDFTLKISRVEAEDVGVYYCVQVSSFPYTFGQGTKVEIKTVAAPSVFIFPPSDEQLKSGTASVVCLLNNFYPREAKVQWKVDNALQSGNSQESVTEQDSKDSTYSLSSTLTLSKADYEKHKVYACEVTHQGLSSPVTKSFNRGEC

SEQ ID NO: 122 - DNA, 654 bp, synthetic construct
  source 1..654: mol_type = other DNA; note = anti-GPC3 light chain; note (original language) = 抗GPC3轻链
gatattgtgctgacgcagtctccactctcactgaccgtcacccctggagagccggcctccatctcctgcaggtctagtgaaagcctcgtacacagtaatggaaacacctacttgagttggcttcagcagaggccaggccagcctccaagactcctaatttataagatttctaaccggttctctggggtcccagacagattcagtggcagtggggcagggacagatttcacactgaaaatcagcagggtggaagctgaggatgtcggggtttattactgcgttcaggtgtcgtcgtttccgtacacttttggccaggggaccaaggtggagatcaaaactgtcgcagctccatccgtgttcatctttccaccctccgacgagcaactgaaaagtggcacagcctccgtcgtctgtctgctgaacaatttctaccctcgggaggccaaggtccagtggaaggtggacaacgctctccagagtggaaatagccaagagtccgttactgagcaggactctaaggattcaacctacagcctctccagcaccctgactctgagcaaggcagattatgagaagcacaaagtctacgcatgtgaagtgactcatcagggactcagctcacccgttaccaagtctttcaacaggggagagtgt

SEQ ID NO: 123 - protein, 445 aa, synthetic construct
  source 1..445: note = anti-GPC3 heavy chain; note (original language) = 抗GPC3重链
QVQLVQSGAEVKKPGASVKLSCKASGYTFTDYEMHWVKQTPGKGLKWIGALDPKTGDTAYAQKFQGRATLTADTSTDTAYMELSSLRSEDSAVYYCTRFYSYTYWGQGTLVTVSSASTKGPSVFPLAPSSKSTSGGTAALGCLVKDYFPEPVTVSWNSGALTSGVHTFPAVLQSSGLYSLSSVVTVPSSSLGTQTYICNVNHKPSNTKVDKKVEPKSCDKTHTCPPCPAPEAAGGPSVFLFPPKPKDTLMISRTPEVTCVVVDVSHEDPEVKFNWYVDGVEVHNAKTKPREEQYNSTYRVVSVLTVLHQDWLNGKEYKCKVSNKALPAPIEKTISKAKGQPREPQVYTLPPSREEMTKNQVSLTCLVKGFYPSDIAVEWESNGQPENNYKTDDDVLDSDGSFFLYSKLTVDKSRWQQGNVFSCSVMHEALHNHYTQKSLSLSPGK

SEQ ID NO: 124 - DNA, 1335 bp, synthetic construct
  source 1..1335: mol_type = other DNA; note = anti-GPC3 heavy chain; note (original language) = 抗GPC3重链
caagtgcaactcgttcaatcaggagctgaggtgaagaaacctggagcatctgtcaagctctcctgtaaggcctccggatacacctttaccgattacgagatgcactgggtgaagcagactcctggaaagggtctgaagtggatcggcgccctggaccctaagaccggagacaccgcttatgcccagaagtttcagggaagagccactctgaccgctgacacatcaaccgataccgcttacatggagctcagctccctgcgcagtgaggattctgctgtgtactattgtacacgcttttatagctacacctactggggacagggcactctcgtgaccgtctcctccgctagcaccaagggcccatcggtcttccccctggcaccctcctccaagagcacctctgggggcacagcggccctgggctgcctggtcaaggactacttccccgaaccggtgacggtgtcgtggaactcaggcgccctgaccagcggcgtgcacaccttcccggctgtcctacagtcctcaggactctactccctcagcagcgtggtgaccgtgccctccagcagcttgggcacccagacctacatctgcaacgtgaatcacaagcccagcaacaccaaggtggacaagaaagttgagcccaaatcttgtgacaaaactcacacatgcccaccgtgcccagcacctgaagccgcagggggaccgtcagtcttcctcttccccccaaaacccaaggacaccctcatgatctcccggacccctgaggtcacatgcgtggtggtggacgtgagccacgaagaccctgaggtcaagttcaactggtacgtggacggcgtggaggtgcataatgccaagacaaagccgcgggaggagcagtacaacagcacgtaccgtgtggtcagcgtcctcaccgtcctgcaccaggactggctgaatggcaaggagtacaagtgcaaggtctccaacaaagccctcccagcccccatcgagaaaaccatctccaaagccaaagggcagccccgagaaccacaggtgtacaccctgcccccatcccgggaggagatgaccaagaaccaggtcagcctgacctgcctggtcaaaggcttctatcccagcgacatcgccgtggagtgggagagcaatgggcagccggagaacaactacaagaccgacgatgacgtgctggactccgacggctccttcttcctctacagcaagctcaccgtggacaagagcaggtggcagcaggggaacgtcttctcatgctccgtgatgcatgaggctctgcacaaccactacacgcagaagagcctctccctgtctccgggtaaa

SEQ ID NO: 125 - protein, 20 aa, synthetic construct
  source 1..20: note = human interleukin-2 signal peptide; note (original language) = 人白介素-2信号肽
MYRMQLLSCIALSLALVTNS

SEQ ID NO: 126 - DNA, 60 bp, synthetic construct
  source 1..60: mol_type = other DNA; note = human interleukin-2 signal peptide; note (original language) = 人白介素-2信号肽
atgtacaggatgcaactcctgtcttgcattgcactaagtcttgcacttgtcacgaattcg

SEQ ID NO: 127 - protein, 216 aa, synthetic construct
  source 1..216: note = CD3 light chain of MutA; note (original language) = MutA的CD3轻链
DIQMTQEPSLTTSPGGTVTLTCRSSTGAVTTSNYANWVQEKPGQAPRGLIGGTNKRAPGTPARFSGSLIGGKAALTITGVQPEDEAIYFCALWYSNLWVFGGGTKLEIKRTVAAPSVFIFPPSDEQLKSGTASVVCLLNNFYPREAKVQWKVDNALQSGNSQESVTEQDSKDSTYALESALTLSKADYEKHKVYACEVTHQGLSSPVTKSFNRGEC

SEQ ID NO: 128 - DNA, 648 bp, synthetic construct
  source 1..648: mol_type = other DNA; note = CD3 light chain of MutA; note (original language) = MutA的CD3轻链
gatattcagatgacacaagaaccaagtctcactacaagccctggaggcaccgttacactgacctgtcgctcttccactggcgccgtgaccacttccaactatgcaaactgggtgcaggagaaacctggacaggctcctagaggtctgattggaggcactaacaagagagctccagggactcctgccaggttcagcggatctctgatcggtgggaaggcagctctgacaatcactggagtgcaacccgaggatgaggctatctacttctgtgctctctggtactcaaatctgtgggtgttcggaggtggaacaaagctggagatcaagcggactgtcgcagctccatccgtgttcatctttccaccctccgacgagcaactgaaaagtggcacagcctccgtcgtctgtctgctgaacaatttctaccctcgggaggccaaggtccagtggaaggtggacaacgctctccagagtggaaatagccaagagtccgttactgagcaggactctaaggattcaacctacgcactcgagagcgctctgactctgagcaaggcagattatgagaagcacaaagtctacgcatgtgaagtgactcatcagggactcagctcacccgttaccaagtctttcaacaggggagagtgt

SEQ ID NO: 129 - protein, 455 aa, synthetic construct
  source 1..455: note = CD3 heavy chain of MutA; note (original language) = MutA的CD3重链
EVQLVESGGGLVQPGGSLKLSCAASGFTFNTYAMNWVRQAPGKGLEWVARIRSKYNNYATYYADSVKDRFTISRDDSKNTAYLQMNNLKTEDTAMYYCVRHGNFGHSYVSWFAYWGQGTLVTVSSASTKGPSVFPLAPSSKSTSGGTAALGCLVKDYFPEPVTVSWNSGALTSGVHTFPAVLQSSGLYTLYSFVTVPSSSLGTQTYICNVNHKPSNTKVDKKVEPKSCDKTHTCPPCPAPEAAGGPSVFLFPPKPKDTLMISRTPEVTCVVVDVSHEDPEVKFNWYVDGVEVHNAKTKPREEQYNSTYRVVSVLTVLHQDWLNGKEYKCKVSNKALPAPIEKTISKAKGQPREPQVYTLPPSREEMTKNQVSLTCLVKGFYPSDIAVEWESNGQPENNYKTTKKKLDSDGSFFLYSKLTVDKSRWQQGNVFSCSVMHEALHNHYTQKSLSLSPGK

SEQ ID NO: 130 - DNA, 1365 bp, synthetic construct
  source 1..1365: mol_type = other DNA; note = CD3 heavy chain of MutA; note (original language) = MutA的CD3重链
gaagtgcaactggttgaaagcggtggaggactggttcagcctggaggctccctcaaactcagttgcgccgcttccggttttacattcaacacttatgccatgaattgggtgcgccaggctcccggaaaaggcctggaatgggtggcacggatcaggagcaaatacaacaattacgccacatattacgctgactccgttaaagacagattcacaatttccagagatgattccaagaatactgcttatctccagatgaacaacctgaagacagaggatacagctatgtactattgcgtgcggcatggcaatttcggacattcctatgtgagttggtttgcctactggggacagggaactctcgttactgtcagctccgctagcaccaagggcccatcggtcttccccctggcaccctcctccaagagcacctctgggggcacagcggccctgggctgcctggtcaaggactacttccccgaaccggtgacggtgtcgtggaactcaggcgccctgaccagcggcgtgcacaccttcccggctgtcctacagtcctcaggactctacacgctctatagctttgtgaccgtgccctccagcagcttgggcacccagacctacatctgcaacgtgaatcacaagcccagcaacaccaaggtggacaagaaagttgagcccaaatcttgtgacaaaactcacacatgcccaccgtgcccagcacctgaagccgcagggggaccgtcagtcttcctcttccccccaaaacccaaggacaccctcatgatctcccggacccctgaggtcacatgcgtggtggtggacgtgagccacgaagaccctgaggtcaagttcaactggtacgtggacggcgtggaggtgcataatgccaagacaaagccgcgggaggagcagtacaacagcacgtaccgtgtggtcagcgtcctcaccgtcctgcaccaggactggctgaatggcaaggagtacaagtgcaaggtctccaacaaagccctcccagcccccatcgagaaaaccatctccaaagccaaagggcagccccgagaaccacaggtgtacaccctgcccccatcccgggaggagatgaccaagaaccaggtcagcctgacctgcctggtcaaaggcttctatcccagcgacatcgccgtggagtgggagagcaatgggcagccggagaacaactacaagaccacgaagaagaagctggactccgacggctccttcttcctctacagcaagctcaccgtggacaagagcaggtggcagcaggggaacgtcttctcatgctccgtgatgcatgaggctctgcacaaccactacacgcagaagagcctctccctgtctccgggtaaa

SEQ ID NO: 131 - protein, 218 aa, synthetic construct
  source 1..218: note = GPC3 light chain of MutA; note (original language) = MutA的GPC3轻链
DIVLTQSPLSLTVTPGEPASISCRSSESLVHSNGNTYLSWLQQRPGQPPRLLIYKISNRFSGVPDRFSGSGAGTDFTLKISRVEAEDVGVYYCVQVSSFPYTFGQGTKVEIKTVAAPSVFIFPPSDEQLKSGTASVVCLLNNFYPREAKVQWKVDNALQSGNSQESVTEQDSKDSTYRLHSVLTLSKADYEKHKVYACEVTHQGLSSPVTKSFNRGEC

SEQ ID NO: 132 - DNA, 654 bp, synthetic construct
  source 1..654: mol_type = other DNA; note = GPC3 light chain of MutA; note (original language) = MutA的GPC3轻链
gatattgtgctgacgcagtctccactctcactgaccgtcacccctggagagccggcctccatctcctgcaggtctagtgaaagcctcgtacacagtaatggaaacacctacttgagttggcttcagcagaggccaggccagcctccaagactcctaatttataagatttctaaccggttctctggggtcccagacagattcagtggcagtggggcagggacagatttcacactgaaaatcagcagggtggaagctgaggatgtcggggtttattactgcgttcaggtgtcgtcgtttccgtacacttttggccaggggaccaaggtggagatcaaaactgtcgcagctccatccgtgttcatctttccaccctccgacgagcaactgaaaagtggcacagcctccgtcgtctgtctgctgaacaatttctaccctcgggaggccaaggtccagtggaaggtggacaacgctctccagagtggaaatagccaagagtccgttactgagcaggactctaaggattcaacctacaggctccatagcgttctgactctgagcaaggcagattatgagaagcacaaagtctacgcatgtgaagtgactcatcagggactcagctcacccgttaccaagtctttcaacaggggagagtgt

SEQ ID NO: 133 - protein, 445 aa, synthetic construct
  source 1..445: note = GPC3 heavy chain of MutA; note (original language) = MutA的GPC3重链
QVQLVQSGAEVKKPGASVKLSCKASGYTFTDYEMHWVKQTPGKGLKWIGALDPKTGDTAYAQKFQGRATLTADTSTDTAYMELSSLRSEDSAVYYCTRFYSYTYWGQGTLVTVSSASTKGPSVFPLAPSSKSTSGGTAALGCLVKDYFPEPVTVSWNSGALTSGVHTFPAVLQSSGLYMLISWVTVPSSSLGTQTYICNVNHKPSNTKVDKKVEPKSCDKTHTCPPCPAPEAAGGPSVFLFPPKPKDTLMISRTPEVTCVVVDVSHEDPEVKFNWYVDGVEVHNAKTKPREEQYNSTYRVVSVLTVLHQDWLNGKEYKCKVSNKALPAPIEKTISKAKGQPREPQVYTLPPSREEMTKNQVSLTCLVKGFYPSDIAVEWESNGQPENNYKTDDDVLDSDGSFFLYSKLTVDKSRWQQGNVFSCSVMHEALHNHYTQKSLSLSPGK

SEQ ID NO: 134 - DNA, 1335 bp, synthetic construct
  source 1..1335: mol_type = other DNA; note = GPC3 heavy chain of MutA; note (original language) = MutA的GPC3重链
caagtgcaactcgttcaatcaggagctgaggtgaagaaacctggagcatctgtcaagctctcctgtaaggcctccggatacacctttaccgattacgagatgcactgggtgaagcagactcctggaaagggtctgaagtggatcggcgccctggaccctaagaccggagacaccgcttatgcccagaagtttcagggaagagccactctgaccgctgacacatcaaccgataccgcttacatggagctcagctccctgcgcagtgaggattctgctgtgtactattgtacacgcttttatagctacacctactggggacagggcactctcgtgaccgtctcctccgctagcaccaagggcccatcggtcttccccctggcaccctcctccaagagcacctctgggggcacagcggccctgggctgcctggtcaaggactacttccccgaaccggtgacggtgtcgtggaactcaggcgccctgaccagcggcgtgcacaccttcccggctgtcctacagtcctcaggactctacatgctcattagctgggtgaccgtgccctccagcagcttgggcacccagacctacatctgcaacgtgaatcacaagcccagcaacaccaaggtggacaagaaagttgagcccaaatcttgtgacaaaactcacacatgcccaccgtgcccagcacctgaagccgcagggggaccgtcagtcttcctcttccccccaaaacccaaggacaccctcatgatctcccggacccctgaggtcacatgcgtggtggtggacgtgagccacgaagaccctgaggtcaagttcaactggtacgtggacggcgtggaggtgcataatgccaagacaaagccgcgggaggagcagtacaacagcacgtaccgtgtggtcagcgtcctcaccgtcctgcaccaggactggctgaatggcaaggagtacaagtgcaaggtctccaacaaagccctcccagcccccatcgagaaaaccatctccaaagccaaagggcagccccgagaaccacaggtgtacaccctgcccccatcccgggaggagatgaccaagaaccaggtcagcctgacctgcctggtcaaaggcttctatcccagcgacatcgccgtggagtgggagagcaatgggcagccggagaacaactacaagaccgacgatgacgtgctggactccgacggctccttcttcctctacagcaagctcaccgtggacaagagcaggtggcagcaggggaacgtcttctcatgctccgtgatgcatgaggctctgcacaaccactacacgcagaagagcctctccctgtctccgggtaaa

SEQ ID NO: 135 - protein, 216 aa, synthetic construct
  source 1..216: note = CD3 light chain of MutB; note (original language) = MutB的CD3轻链
DIQMTQEPSLTTSPGGTVTLTCRSSTGAVTTSNYANWVQEKPGQAPRGLIGGTNKRAPGTPARFSGSLIGGKAALTITGVQPEDEAIYFCALWYSNLWVFGGGTKLEIKRTVAAPSVFIFPPSDEQLKSGTASVVCLLNNFYPREAKVQWKVDNALQSGNSQESVTEQDSKDSTYRLWSLLTLSKADYEKHKVYACEVTHQGLSSPVTKSFNRGEC

SEQ ID NO: 136 - DNA, 648 bp, synthetic construct
  source 1..648: mol_type = other DNA; note = CD3 light chain of MutB; note (original language) = MutB的CD3轻链
gatattcagatgacacaagaaccaagtctcactacaagccctggaggcaccgttacactgacctgtcgctcttccactggcgccgtgaccacttccaactatgcaaactgggtgcaggagaaacctggacaggctcctagaggtctgattggaggcactaacaagagagctccagggactcctgccaggttcagcggatctctgatcggtgggaaggcagctctgacaatcactggagtgcaacccgaggatgaggctatctacttctgtgctctctggtactcaaatctgtgggtgttcggaggtggaacaaagctggagatcaagcggactgtcgcagctccatccgtgttcatctttccaccctccgacgagcaactgaaaagtggcacagcctccgtcgtctgtctgctgaacaatttctaccctcgggaggccaaggtccagtggaaggtggacaacgctctccagagtggaaatagccaagagtccgttactgagcaggactctaaggattcaacctaccgtctctggagccttctgactctgagcaaggcagattatgagaagcacaaagtctacgcatgtgaagtgactcatcagggactcagctcacccgttaccaagtctttcaacaggggagagtgt

SEQ ID NO: 137 - protein, 455 aa, synthetic construct
  source 1..455: note = CD3 heavy chain of MutB; note (original language) = MutB的CD3重链
EVQLVESGGGLVQPGGSLKLSCAASGFTFNTYAMNWVRQAPGKGLEWVARIRSKYNNYATYYADSVKDRFTISRDDSKNTAYLQMNNLKTEDTAMYYCVRHGNFGHSYVSWFAYWGQGTLVTVSSASTKGPSVFPLAPSSKSTSGGTAALGCLVKDYFPEPVTVSWNSGALTSGVHTFPAVLQSSGLYVLLSMVTVPSSSLGTQTYICNVNHKPSNTKVDKKVEPKSCDKTHTCPPCPAPEAAGGPSVFLFPPKPKDTLMISRTPEVTCVVVDVSHEDPEVKFNWYVDGVEVHNAKTKPREEQYNSTYRVVSVLTVLHQDWLNGKEYKCKVSNKALPAPIEKTISKAKGQPREPQVYTLPPSREEMTKNQVSLTCLVKGFYPSDIAVEWESNGQPENNYKTTKKKLDSDGSFFLYSKLTVDKSRWQQGNVFSCSVMHEALHNHYTQKSLSLSPGK

SEQ ID NO: 138 - DNA, 1365 bp, synthetic construct
  source 1..1365: mol_type = other DNA; note = CD3 heavy chain of MutB; note (original language) = MutB的CD3重链
gaagtgcaactggttgaaagcggtggaggactggttcagcctggaggctccctcaaactcagttgcgccgcttccggttttacattcaacacttatgccatgaattgggtgcgccaggctcccggaaaaggcctggaatgggtggcacggatcaggagcaaatacaacaattacgccacatattacgctgactccgttaaagacagattcacaatttccagagatgattccaagaatactgcttatctccagatgaacaacctgaagacagaggatacagctatgtactattgcgtgcggcatggcaatttcggacattcctatgtgagttggtttgcctactggggacagggaactctcgttactgtcagctccgctagcaccaagggcccatcggtcttccccctggcaccctcctccaagagcacctctgggggcacagcggccctgggctgcctggtcaaggactacttccccgaaccggtgacggtgtcgtggaactcaggcgccctgaccagcggcgtgcacaccttcccggctgtcctacagtcctcaggactctacgtgctcttgagcatggtgaccgtgccctccagcagcttgggcacccagacctacatctgcaacgtgaatcacaagcccagcaacaccaaggtggacaagaaagttgagcccaaatcttgtgacaaaactcacacatgcccaccgtgcccagcacctgaagccgcagggggaccgtcagtcttcctcttccccccaaaacccaaggacaccctcatgatctcccggacccctgaggtcacatgcgtggtggtggacgtgagccacgaagaccctgaggtcaagttcaactggtacgtggacggcgtggaggtgcataatgccaagacaaagccgcgggaggagcagtacaacagcacgtaccgtgtggtcagcgtcctcaccgtcctgcaccaggactggctgaatggcaaggagtacaagtgcaaggtctccaacaaagccctcccagcccccatcgagaaaaccatctccaaagccaaagggcagccccgagaaccacaggtgtacaccctgcccccatcccgggaggagatgaccaagaaccaggtcagcctgacctgcctggtcaaaggcttctatcccagcgacatcgccgtggagtgggagagcaatgggcagccggagaacaactacaagaccacgaagaagaagctggactccgacggctccttcttcctctacagcaagctcaccgtggacaagagcaggtggcagcaggggaacgtcttctcatgctccgtgatgcatgaggctctgcacaaccactacacgcagaagagcctctccctgtctccgggtaaa

SEQ ID NO: 139 - protein, 218 aa, synthetic construct; identical to SEQ ID NO: 121
  source 1..218: note = GPC3 light chain of MutB; note (original language) = MutB的GPC3轻链

SEQ ID NO: 140 - DNA, 654 bp, synthetic construct; identical to SEQ ID NO: 122
  source 1..654: mol_type = other DNA; note = GPC3 light chain of MutB; note (original language) = MutB的GPC3轻链

SEQ ID NO: 141 - protein, 445 aa, synthetic construct
  source 1..445: note = GPC3 heavy chain of MutB; note (original language) = MutB的GPC3重链
QVQLVQSGAEVKKPGASVKLSCKASGYTFTDYEMHWVKQTPGKGLKWIGALDPKTGDTAYAQKFQGRATLTADTSTDTAYMELSSLRSEDSAVYYCTRFYSYTYWGQGTLVTVSSASTKGPSVFPLAPSSKSTSGGTAALGCLVKDYFPEPVTVSWNSGALTSGVHTFPAVLQSSGLYTLRSFVTVPSSSLGTQTYICNVNHKPSNTKVDKKVEPKSCDKTHTCPPCPAPEAAGGPSVFLFPPKPKDTLMISRTPEVTCVVVDVSHEDPEVKFNWYVDGVEVHNAKTKPREEQYNSTYRVVSVLTVLHQDWLNGKEYKCKVSNKALPAPIEKTISKAKGQPREPQVYTLPPSREEMTKNQVSLTCLVKGFYPSDIAVEWESNGQPENNYKTDDDVLDSDGSFFLYSKLTVDKSRWQQGNVFSCSVMHEALHNHYTQKSLSLSPGK

SEQ ID NO: 142 - DNA, 1335 bp, synthetic construct
  source 1..1335: mol_type = other DNA; note = GPC3 heavy chain of MutB; note (original language) = MutB的GPC3重链
caagtgcaactcgttcaatcaggagctgaggtgaagaaacctggagcatctgtcaagctctcctgtaaggcctccggatacacctttaccgattacgagatgcactgggtgaagcagactcctggaaagggtctgaagtggatcggcgccctggaccctaagaccggagacaccgcttatgcccagaagtttcagggaagagccactctgaccgctgacacatcaaccgataccgcttacatggagctcagctccctgcgcagtgaggattctgctgtgtactattgtacacgcttttatagctacacctactggggacagggcactctcgtgaccgtctcctccgctagcaccaagggcccatcggtcttccccctggcaccctcctccaagagcacctctgggggcacagcggccctgggctgcctggtcaaggactacttccccgaaccggtgacggtgtcgtggaactcaggcgccctgaccagcggcgtgcacaccttcccggctgtcctacagtcctcaggactctacacgctccgtagctttgtgaccgtgccctccagcagcttgggcacccagacctacatctgcaacgtgaatcacaagcccagcaacaccaaggtggacaagaaagttgagcccaaatcttgtgacaaaactcacacatgcccaccgtgcccagcacctgaagccgcagggggaccgtcagtcttcctcttccccccaaaacccaaggacaccctcatgatctcccggacccctgaggtcacatgcgtggtggtggacgtgagccacgaagaccctgaggtcaagttcaactggtacgtggacggcgtggaggtgcataatgccaagacaaagccgcgggaggagcagtacaacagcacgtaccgtgtggtcagcgtcctcaccgtcctgcaccaggactggctgaatggcaaggagtacaagtgcaaggtctccaacaaagccctcccagcccccatcgagaaaaccatctccaaagccaaagggcagccccgagaaccacaggtgtacaccctgcccccatcccgggaggagatgaccaagaaccaggtcagcctgacctgcctggtcaaaggcttctatcccagcgacatcgccgtggagtgggagagcaatgggcagccggagaacaactacaagaccgacgatgacgtgctggactccgacggctccttcttcctctacagcaagctcaccgtggacaagagcaggtggcagcaggggaacgtcttctcatgctccgtgatgcatgaggctctgcacaaccactacacgcagaagagcctctccctgtctccgggtaaa

SEQ ID NO: 143 - protein, 216 aa, synthetic construct
  source 1..216: note = CD3 light chain of MutA+D-D; note (original language) = MutA+D-D的CD3轻链
DIQMTQEPSLTTSPGGTVTLTCRSSTGAVTTSNYANWVQEKPGQAPRGLIGGTNKRAPGTPARFSGSLIGGKAALTITGVQPEDEAIYFCALWYSNLWVFGGGTKLEIKRTVAAPSVFIFPPSDEQLKSGTASVVCLLNNFYPREAKVQWKVDNALQSGNSQESVTEQDSKDSTYALESDLTLSKADYEKHKVYACEVTHQGLSSPVTKSFNRGEC

SEQ ID NO: 144 - DNA, 648 bp, synthetic construct
  source 1..648: mol_type = other DNA; note = CD3 light chain of MutA+D-D; note (original language) = MutA+D-D的CD3轻链
gatattcagatgacacaagaaccaagtctcactacaagccctggaggcaccgttacactgacctgtcgctcttccactggcgccgtgaccacttccaactatgcaaactgggtgcaggagaaacctggacaggctcctagaggtctgattggaggcactaacaagagagctccagggactcctgccaggttcagcggatctctgatcggtgggaaggcagctctgacaatcactggagtgcaacccgaggatgaggctatctacttctgtgctctctggtactcaaatctgtgggtgttcggaggtggaacaaagctggagatcaagcggactgtcgcagctccatccgtgttcatctttccaccctccgacgagcaactgaaaagtggcacagcctccgtcgtctgtctgctgaacaatttctaccctcgggaggccaaggtccagtggaaggtggacaacgctctccagagtggaaatagccaagagtccgttactgagcaggactctaaggattcaacctacgctctcgagagcgatctgactctgagcaaggcagattatgagaagcacaaagtctacgcatgtgaagtgactcatcagggactcagctcacccgttaccaagtctttcaacaggggagagtgt

SEQ ID NO: 145 - protein, 455 aa, synthetic construct; identical to SEQ ID NO: 129
  source 1..455: note = CD3 heavy chain of MutA+D-D; note (original language) = MutA+D-D的CD3重链

SEQ ID NO: 146 - DNA, 1365 bp, synthetic construct; identical to SEQ ID NO: 130
  source 1..1365: mol_type = other DNA; note = CD3 heavy chain of MutA+D-D; note (original language) = MutA+D-D的CD3重链

SEQ ID NO: 147 - protein, 218 aa, synthetic construct; identical to SEQ ID NO: 131
  source 1..218: note = GPC3 light chain of MutA+D-D; note (original language) = MutA+D-D的GPC3轻链

SEQ ID NO: 148 - DNA, 654 bp, synthetic construct; identical to SEQ ID NO: 132
  source 1..654: mol_type = other DNA; note = GPC3 light chain of MutA+D-D; note (original language) = MutA+D-D的GPC3轻链

SEQ ID NO: 149 - protein, 445 aa, synthetic construct
  source 1..445: note = GPC3 heavy chain of MutA+D-D; note (original language) = MutA+D-D的GPC3重链
QVQLVQSGAEVKKPGASVKLSCKASGYTFTDYEMHWVKQTPGKGLKWIGALDPKTGDTAYAQKFQGRATLTADTSTDTAYMELSSLRSEDSAVYYCTRFYSYTYWGQGTLVTVSSASTKGPSVFPLAPSSKSTSGGTAALGCLVKDYFPEPVTVSWNSGALTSGVHTFPAVLQSSGLYMLDSWVTVPSSSLGTQTYICNVNHKPSNTKVDKKVEPKSCDKTHTCPPCPAPEAAGGPSVFLFPPKPKDTLMISRTPEVTCVVVDVSHEDPEVKFNWYVDGVEVHNAKTKPREEQYNSTYRVVSVLTVLHQDWLNGKEYKCKVSNKALPAPIEKTISKAKGQPREPQVYTLPPSREEMTKNQVSLTCLVKGFYPSDIAVEWESNGQPENNYKTDDDVLDSDGSFFLYSKLTVDKSRWQQGNVFSCSVMHEALHNHYTQKSLSLSPGK

SEQ ID NO: 150 - DNA, 1335 bp, synthetic construct
  source 1..1335: mol_type = other DNA; note = GPC3 heavy chain of MutA+D-D; note (original language) = MutA+D-D的GPC3重链
caagtgcaactcgttcaatcaggagctgaggtgaagaaacctggagcatctgtcaagctctcctgtaaggcctccggatacacctttaccgattacgagatgcactgggtgaagcagactcctggaaagggtctgaagtggatcggcgccctggaccctaagaccggagacaccgcttatgcccagaagtttcagggaagagccactctgaccgctgacacatcaaccgataccgcttacatggagctcagctccctgcgcagtgaggattctgctgtgtactattgtacacgcttttatagctacacctactggggacagggcactctcgtgaccgtctcctccgctagcaccaagggcccatcggtcttccccctggcaccctcctccaagagcacctctgggggcacagcggccctgggctgcctggtcaaggactacttccccgaaccggtgacggtgtcgtggaactcaggcgccctgaccagcggcgtgcacaccttcccggctgtcctacagtcctcaggactctacatgctcgacagctgggtgaccgtgccctccagcagcttgggcacccagacctacatctgcaacgtgaatcacaagcccagcaacaccaaggtggacaagaaagttgagcccaaatcttgtgacaaaactcacacatgcccaccgtgcccagcacctgaagccgcagggggaccgtcagtcttcctcttccccccaaaacccaaggacaccctcatgatctcccggacccctgaggtcacatgcgtggtggtggacgtgagccacgaagaccctgaggtcaagttcaactggtacgtggacggcgtggaggtgcataatgccaagacaaagccgcgggaggagcagtacaacagcacgtaccgtgtggtcagcgtcctcaccgtcctgcaccaggactggctgaatggcaaggagtacaagtgcaaggtctccaacaaagccctcccagcccccatcgagaaaaccatctccaaagccaaagggcagccccgagaaccacaggtgtacaccctgcccccatcccgggaggagatgaccaagaaccaggtcagcctgacctgcctggtcaaaggcttctatcccagcgacatcgccgtggagtgggagagcaatgggcagccggagaacaactacaagaccgacgatgacgtgctggactccgacggctccttcttcctctacagcaagctcaccgtggacaagagcaggtggcagcaggggaacgtcttctcatgctccgtgatgcatgaggctctgcacaaccactacacgcagaagagcctctccctgtctccgggtaaa

SEQ ID NO: 151 - protein, 216 aa, synthetic construct
  source 1..216: note = CD3 light chain of MutB+K-K; note (original language) = MutB+K-K的CD3轻链
DIQMTQEPSLTTSPGGTVTLTCRSSTGAVTTSNYANWVQEKPGQAPRGLIGGTNKRAPGTPARFSGSLIGGKAALTITGVQPEDEAIYFCALWYSNLWVFGGGTKLEIKRTVAAPSVFIFPPSDEQLKSGTASVVCLLNNFYPREAKVQWKVDNALQSGNSQESVTEQDSKDSTYRLWSKLTLSKADYEKHKVYACEVTHQGLSSPVTKSFNRGEC

SEQ ID NO: 152 - DNA, 648 bp, synthetic construct
  source 1..648: mol_type = other DNA; note = CD3 light chain of MutB+K-K; note (original language) = MutB+K-K的CD3轻链
gatattcagatgacacaagaaccaagtctcactacaagccctggaggcaccgttacactgacctgtcgctcttccactggcgccgtgaccacttccaactatgcaaactgggtgcaggagaaacctggacaggctcctagaggtctgattggaggcactaacaagagagctccagggactcctgccaggttcagcggatctctgatcggtgggaaggcagctctgacaatcactggagtgcaacccgaggatgaggctatctacttctgtgctctctggtactcaaatctgtgggtgttcggaggtggaacaaagctggagatcaagcggactgtcgcagctccatccgtgttcatctttccaccctccgacgagcaactgaaaagtggcacagcctccgtcgtctgtctgctgaacaatttctaccctcgggaggccaaggtccagtggaaggtggacaacgctctccagagtggaaatagccaagagtccgttactgagcaggactctaaggattcaacctaccgtctctggagcaagctgactctgagcaaggcagattatgagaagcacaaagtctacgcatgtgaagtgactcatcagggactcagctcacccgttaccaagtctttcaacaggggagagtgt

SEQ ID NO: 153 - protein, 455 aa, synthetic construct; identical to SEQ ID NO: 137
  source 1..455: note = CD3 heavy chain of MutB+K-K; note (original language) = MutB+K-K的CD3重链

SEQ ID NO: 154 - DNA, 1365 bp, synthetic construct; identical to SEQ ID NO: 138
  source 1..1365: mol_type = other DNA; note = CD3 heavy chain of MutB+K-K; note (original language) = MutB+K-K的CD3重链

SEQ ID NO: 155 - protein, 218 aa, synthetic construct; identical to SEQ ID NO: 121
  source 1..218: note = GPC3 light chain of MutB+K-K; note (original language) = MutB+K-K的GPC3轻链

SEQ ID NO: 156 - DNA, 654 bp, synthetic construct; identical to SEQ ID NO: 122
  source 1..654: mol_type = other DNA; note = GPC3 light chain of MutB+K-K; note (original language) = MutB+K-K的GPC3轻链

SEQ ID NO: 157 - protein, 445 aa, synthetic construct
  source 1..445: note = GPC3 heavy chain of MutB+K-K; note (original language) = MutB+K-K的GPC3重链
QVQLVQSGAEVKKPGASVKLSCKASGYTFTDYEMHWVKQTPGKGLKWIGALDPKTGDTAYAQKFQGRATLTADTSTDTAYMELSSLRSEDSAVYYCTRFYSYTYWGQGTLVTVSSASTKGPSVFPLAPSSKSTSGGTAALGCLVKDYFPEPVTVSWNSGALTSGVHTFPAVLQSSGLYTLRSFVKVPSSSLGTQTYICNVNHKPSNTKVDKKVEPKSCDKTHTCPPCPAPEAAGGPSVFLFPPKPKDTLMISRTPEVTCVVVDVSHEDPEVKFNWYVDGVEVHNAKTKPREEQYNSTYRVVSVLTVLHQDWLNGKEYKCKVSNKALPAPIEKTISKAKGQPREPQVYTLPPSREEMTKNQVSLTCLVKGFYPSDIAVEWESNGQPENNYKTDDDVLDSDGSFFLYSKLTVDKSRWQQGNVFSCSVMHEALHNHYTQKSLSLSPGK

SEQ ID NO: 158 - DNA, 1335 bp, synthetic construct
  source 1..1335: mol_type = other DNA; note = GPC3 heavy chain of MutB+K-K; note (original language) = MutB+K-K的GPC3重链
caagtgcaactcgttcaatcaggagctgaggtgaagaaacctggagcatctgtcaagctctcctgtaaggcctccggatacacctttaccgattacgagatgcactgggtgaagcagactcctggaaagggtctgaagtggatcggcgccctggaccctaagaccggagacaccgcttatgcccagaagtttcagggaagagccactctgaccgctgacacatcaaccgataccgcttacatggagctcagctccctgcgcagtgaggattctgctgtgtactattgtacacgcttttatagctacacctactggggacagggcactctcgtgaccgtctcctccgctagcaccaagggcccatcggtcttccccctggcaccctcctccaagagcacctctgggggcacagcggccctgggctgcctggtcaaggactacttccccgaaccggtgacggtgtcgtggaactcaggcgccctgaccagcggcgtgcacaccttcccggctgtcctacagtcctcaggactctacacgctccgtagctttgtgaaggtgccctccagcagcttgggcacccagacctacatctgcaacgtgaatcacaagcccagcaacaccaaggtggacaagaaagttgagcccaaatcttgtgacaaaactcacacatgcccaccgtgcccagcacctgaagccgcagggggaccgtcagtcttcctcttccccccaaaacccaaggacaccctcatgatctcccggacccctgaggtcacatgcgtggtggtggacgtgagccacgaagaccctgaggtcaagttcaactggtacgtggacggcgtggaggtgcataatgccaagacaaagccgcgggaggagcagtacaacagcacgtaccgtgtggtcagcgtcctcaccgtcctgcaccaggactggctgaatggcaaggagtacaagtgcaaggtctccaacaaagccctcccagcccccatcgagaaaaccatctccaaagccaaagggcagccccgagaaccacaggtgtacaccctgcccccatcccgggaggagatgaccaagaaccaggtcagcctgacctgcctggtcaaaggcttctatcccagcgacatcgccgtggagtgggagagcaatgggcagccggagaacaactacaagaccgacgatgacgtgctggactccgacggctccttcttcctctacagcaagctcaccgtggacaagagcaggtggcagcaggggaacgtcttctcatgctccgtgatgcatgaggctctgcacaaccactacacgcagaagagcctctccctgtctccgggtaaa

SEQ ID NO: 159 - protein, 242 aa, synthetic construct
  source 1..242: note = ScFv of anti-GPC3; note (original language) = 抗GPC3的ScFv
QVQLVQSGAEVKKPGASVKLSCKASGYTFTDYEMHWVKQTPGKGLKWIGALDPKTGDTAYAQKFQGRATLTADTSTDTAYMELSSLRSEDSAVYYCTRFYSYTYWGQGTLVTVSSGGGGSGGGGSGGGGSDIVLTQSPLSLTVTPGEPASISCRSSESLVHSNGNTYLSWLQQRPGQPPRLLIYKISNRFSGVPDRFSGSGAGTDFTLKISRVEAEDVGVYYCVQVSSFPYTFGQGTKVEIK

SEQ ID NO: 160 - DNA, 726 bp, synthetic construct
  source 1..726: mol_type = other DNA; note = ScFv of anti-GPC3; note (original language) = 抗GPC3的ScFv
caagtgcaactcgttcaatcaggagctgaggtgaagaaacctggagcatctgtcaagctctcctgtaaggcctccggatacacctttaccgattacgagatgcactgggtgaagcagactcctggaaagggtctgaagtggatcggcgccctggaccctaagaccggagacaccgcttatgcccagaagtttcagggaagagccactctgaccgctgacacatcaaccgataccgcttacatggagctcagctccctgcgcagtgaggattctgctgtgtactattgtacacgcttttatagctacacctactggggacagggcactctcgtgaccgtctcctccggtggaggtggatctggcggcggcggctcaggcggaggaggttccgatattgtgctgacgcagtctccactctcactgaccgtcacccctggagagccggcctccatctcctgcaggtctagtgaaagcctcgtacacagtaatggaaacacctacttgagttggcttcagcagaggccaggccagcctccaagactcctaatttataagatttctaaccggttctctggggtcccagacagattcagtggcagtggggcagggacagatttcacactgaaaatcagcagggtggaagctgaggatgtcggggtttattactgcgttcaggtgtcgtcgtttccgtacacttttggccaggggaccaaggtggagatcaaa

SEQ ID NO: 161 - protein, 210 aa, synthetic construct
  source 1..210: note = an Anti-CD3 light chain of a Crossmab-CD3 bispecific antibody; note (original language) = Crossmab-CD3双特异性抗体的抗CD3轻链
DIQMTQEPSLTTSPGGTVTLTCRSSTGAVTTSNYANWVQEKPGQAPRGLIGGTNKRAPGTPARFSGSLIGGKAALTITGVQPEDEAIYFCALWYSNLWVFGGGTKLEIKRSSASTKGPSVFPLAPSSKSTSGGTAALGCLVKDYFPEPVTVSWNSGALTSGVHTFPAVLQSSGLYSLSSVVTVPSSSLGTQTYICNVNHKPSNTKVDKKV

SEQ ID NO: 162 - DNA, 630 bp, synthetic construct
  source 1..630: mol_type = other DNA; note = an Anti-CD3 light chain of a Crossmab-CD3 bispecific antibody; note (original language) = Crossmab-CD3双特异性抗体的抗CD3轻链
gatattcagatgacacaagaaccaagtctcactacaagccctggaggcaccgttacactgacctgtcgctcttccactggcgccgtgaccacttccaactatgcaaactgggtgcaggagaaacctggacaggctcctagaggtctgattggaggcactaacaagagagctccagggactcctgccaggttcagcggatctctgatcggtgggaaggcagctctgacaatcactggagtgcaacccgaggatgaggctatctacttctgtgctctctggtactcaaatctgtgggtgttcggaggtggaacaaagctggagatcaagcggtcttcagctagcaccaagggcccatcggtcttccccctggcaccctcctccaagagcacctctgggggcacagcggccctgggctgcctggtcaaggactacttccccgaaccggtgacggtgtcgtggaactcaggcgccctgaccagcggcgtgcacaccttcccggctgtcctacagtcctcaggactctactccctcagcagcgtggtgaccgtgccctccagcagcttgggcacccagacctacatctgcaacgtgaatcacaagcccagcaacaccaaggtggacaagaaagtt

SEQ ID NO: 163 - protein, 464 aa, synthetic construct
  source 1..464: note = an Anti-CD3 heavy chain of a Crossmab-CD3 bispecific antibody; note (original language) = Crossmab-CD3双特异性抗体的抗CD3重链
EVQLVESGGGLVQPGGSLKLSCAASGFTFNTYAMNWVRQAPGKGLEWVARIRSKYNNYATYYADSVKDRFTISRDDSKNTAYLQMNNLKTEDTAMYYCVRHGNFGTSYVSWFAYWGQGTLVTVSSASVAAPSVFIFPPSDEQLKSGTASVVCLLNNFYPREAKVQWKVDNALQSGNSQESVTEQDSKDSTYSLSSTLTLSKADYEKHKVYACEVTHQGLSSPVTKSFNRGECEPKSCDKTHTCPPCPAPEAAGGPSVFLFPPKPKDTLMISRTPEVTCVVVDVSHEDPEVKFNWYVDGVEVHNAKTKPREEQYNSTYRVVSVLTVLHQDWLNGKEYKCKVSNKALPAPIEKTISKAKGQPREPQVYTLPPSREEMTKNQVSLTCLVKGFYPSDIAVEWESNGQPENNYKTTKKKLDSDGSFFLYSKLTVDKSRWQQGNVFSCSVMHEALHNHYTQKSLSLSPGK

SEQ ID NO: 164 - DNA, 1392 bp, synthetic construct
  source 1..1392: mol_type = other DNA; note = an Anti-CD3 heavy chain of a Crossmab-CD3 bispecific antibody; note (original language) = Crossmab-CD3双特异性抗体的抗CD3重链
gaagtgcaactggttgaaagcggtggaggactggttcagcctggaggctccctcaaactcagttgcgccgcttccggttttacattcaacacttatgccatgaattgggtgcgccaggctcccggaaaaggcctggaatgggtggcacggatcaggagcaaatacaacaattacgccacatattacgctgactccgttaaagacagattcacaatttccagagatgattccaagaatactgcttatctccagatgaacaacctgaagacagaggatacagctatgtactattgcgtgcggcatggcaatttcggaacttcctatgtgagttggtttgcctactggggacagggaactctcgttactgtcagctccgcaagtgtcgcagctccatccgtgttcatctttccaccctccgacgagcaactgaaaagtggcacagcctccgtcgtctgtctgctgaacaatttctaccctcgggaggccaaggtccagtggaaggtggacaacgctctccagagtggaaatagccaagagtccgttactgagcaggactctaaggattcaacctacagcctctccagcaccctgactctgagcaaggcagattatgagaagcacaaagtctacgcatgtgaagtgactcatcagggactcagctcacccgttaccaagtctttcaacaggggagagtgtgagcccaaatcttgtgacaaaactcacacatgcccaccgtgcccagcacctgaagccgcagggggaccgtcagtcttcctcttccccccaaaacccaaggacaccctcatgatctcccggacccctgaggtcacatgcgtggtggtggacgtgagccacgaagaccctgaggtcaagttcaactggtacgtggacggcgtggaggtgcataatgccaagacaaagccgcgggaggagcagtacaacagcacgtaccgtgtggtcagcgtcctcaccgtcctgcaccaggactggctgaatggcaaggagtacaagtgcaaggtctccaacaaagccctcccagcccccatcgagaaaaccatctccaaagccaaagggcagccccgagaaccacaggtgtacaccctgcccccatcccgggaggagatgaccaagaaccaggtcagcctgacctgcctggtcaaaggcttctatcccagcgacatcgccgtggagtgggagagcaatgggcagccggagaacaactacaagaccacgaagaagaagctggactccgacggctccttcttcctctacagcaagctcaccgtggacaagagcaggtggcagcaggggaacgtcttctcatgctccgtgatgcatgaggctctgcacaaccactacacgcagaagagcctctccctgtctccgggtaaa

SEQ ID NO: 165 - protein, 212 aa, synthetic construct
  source 1..212: note = an Anti-GPC3 light chain of a Crossmab-GPC3 bispecific antibody; note (original language) = Crossmab-GPC3双特异性抗体的抗GPC3轻链
DIVLTQSPLSLTVTPGEPASISCRSSESLVHSNGNTYLSWLQQRPGQPPRLLIYKISNRFSGVPDRFSGSGAGTDFTLKISRVEAEDVGVYYCVQVSSFPYTFGQGTKVEIKSSASTKGPSVFPLAPSSKSTSGGTAALGCLVKDYFPEPVTVSWNSGALTSGVHTFPAVLQSSGLYSLSSVVTVPSSSLGTQTYICNVNHKPSNTKVDKKV

SEQ ID NO: 166 - DNA, 636 bp, synthetic construct
  source 1..636: mol_type = other DNA; note = an Anti-GPC3 light chain of a Crossmab-GPC3 bispecific antibody; note (original language) = Crossmab-GPC3双特异性抗体的抗GPC3轻链
gatattgtgctgacgcagtctccactctcactgaccgtcacccctggagagccggcctccatctcctgcaggtctagtgaaagcctcgtacacagtaatggaaacacctacttgagttggcttcagcagaggccaggccagcctccaagactcctaatttataagatttctaaccggttctctggggtcccagacagattcagtggcagtggggcagggacagatttcacactgaaaatcagcagggtggaagctgaggatgtcggggtttattactgcgttcaggtgtcgtcgtttccgtacacttttggccaggggaccaaggtggagatcaaatcttcagctagcaccaagggcccatcggtcttccccctggcaccctcctccaagagcacctctgggggcacagcggccctgggctgcctggtcaaggactacttccccgaaccggtgacggtgtcgtggaactcaggcgccctgaccagcggcgtgcacaccttcccggctgtcctacagtcctcaggactctactccctcagcagcgtggtgaccgtgccctccagcagcttgggcacccagacctacatctgcaacgtgaatcacaagcccagcaacaccaaggtggacaagaaagtt

SEQ ID NO: 167 - protein, 454 aa, synthetic construct
  source 1..454: note = an Anti-GPC3 heavy chain of a Crossmab-GPC3 bispecific antibody; note (original language) = Crossmab-GPC3双特异性抗体的抗GPC3重链
QVQLVQSGAEVKKPGASVKLSCKASGYTFTDYEMHWVKQTPGKGLKWIGALDPKTGDTAYAQKFQGRATLTADTSTDTAYMELSSLRSEDSAVYYCTRFYSYTYWGQGTLVTVSSASVAAPSVFIFPPSDEQLKSGTASVVCLLNNFYPREAKVQWKVDNALQSGNSQESVTEQDSKDSTYSLSSTLTLSKADYEKHKVYACEVTHQGLSSPVTKSFNRGECEPKSCDKTHTCPPCPAPEAAGGPSVFLFPPKPKDTLMISRTPEVTCVVVDVSHEDPEVKFNWYVDGVEVHNAKTKPREEQYNSTYRVVSVLTVLHQDWLNGKEYKCKVSNKALPAPIEKTISKAKGQPREPQVYTLPPSREEMTKNQVSLTCLVKGFYPSDIAVEWESNGQPENNYKTDDDVLDSDGSFFLYSKLTVDKSRWQQGNVFSCSVMHEALHNHYTQKSLSLSPGK

SEQ ID NO: 168 - DNA, 1362 bp, synthetic construct
  source 1..1362: mol_type = other DNA; note = an Anti-GPC3 heavy chain of a Crossmab-GPC3 bispecific antibody; note (original language) = Crossmab-GPC3双特异性抗体的抗GPC3重链
caagtgcaactcgttcaatcaggagctgaggtgaagaaacctggagcatctgtcaagctctcctgtaaggcctccggatacacctttaccgattacgagatgcactgggtgaagcagactcctggaaagggtctgaagtggatcggcgccctggaccctaagaccggagacaccgcttatgcccagaagtttcagggaagagccactctgaccgctgacacatcaaccgataccgcttacatggagctcagctccctgcgcagtgaggattctgctgtgtactattgtacacgcttttatagctacacctactggggacagggcactctcgtgaccgtctcctccgcaagtgtcgcagctccatccgtgttcatctttccaccctccgacgagcaactgaaaagtggcacagcctccgtcgtctgtctgctgaacaatttctaccctcgggaggccaaggtccagtggaaggtggacaacgctctccagagtggaaatagccaagagtccgttactgagcaggactctaaggattcaacctacagcctctccagcaccctgactctgagcaaggcagattatgagaagcacaaagtctacgcatgtgaagtgactcatcagggactcagctcacccgttaccaagtctttcaacaggggagagtgtgagcccaaatcttgtgacaaaactcacacatgcccaccgtgcccagcacctgaagccgcagggggaccgtcagtcttcctcttccccccaaaacccaaggacaccctcatgatctcccggacccctgaggtcacatgcgtggtggtggacgtgagccacgaagaccctgaggtcaagttcaactggtacgtggacggcgtggaggtgcataatgccaagacaaagccgcgggaggagcagtacaacagcacgtaccgtgtggtcagcgtcctcaccgtcctgcaccaggactggctgaatggcaaggagtacaagtgcaaggtctccaacaaagccctcccagcccccatcgagaaaaccatctccaaagccaaagggcagccccgagaaccacaggtgtacaccctgcccccatcccgggaggagatgaccaagaaccaggtcagcctgacctgcctggtcaaaggcttctatcccagcgacatcgccgtggagtgggagagcaatgggcagccggagaacaactacaagaccgacgatgacgtgctggactccgacggctccttcttcctctacagcaagctcaccgtggacaagagcaggtggcagcaggggaacgtcttctcatgctccgtgatgcatgaggctctgcacaaccactacacgcagaagagcctctccctgtctccgggtaaa